European Patent Application EP 4 286 538 A2, published December 6, 2023. Title: PATHOGEN DIAGNOSTIC TEST. Applicant: Octant, Inc. Application EP. The sequence listing filed with the application follows.

SEQUENCE LISTING (632 sequences)

SEQ ID NO: 1 - RNA, 108 nt, synthetic construct
  misc_feature 1..108: note = source = /note="Description of Artificial Sequence: Synthetic polynucleotide"
  source 1..108: mol_type = other RNA
gctggtgctgcagcttattatgtgggtgtgtatctcacgaagcgaccctttggaaaatataatgaaaatggaaccattacagatgctgtagactgtgcacttgaccct

SEQ ID NO: 2 - RNA, 108 nt, synthetic construct
  misc_feature 1..108: note = source = /note="Description of Artificial Sequence: Synthetic polynucleotide"
  source 1..108: mol_type = other RNA
gctggtgctgcagcttattatgtgggtcctcgctaggacgtcgctatgacgccaaaatataatgaaaatggaaccattacagatgctgtagactgtgcacttgaccct

SEQ ID NO: 3 - RNA, 108 nt, synthetic construct
  misc_feature 1..108: note = source = /note="Description of Artificial Sequence: Synthetic polynucleotide"
  source 1..108: mol_type = other RNA
gctggtgctgcagcttattatgtgggtagcacgacttgatctaactgacactaaaaatataatgaaaatggaaccattacagatgctgtagactgtgcacttgaccct

SEQ ID NO: 4 - RNA, 108 nt, synthetic construct
  misc_feature 1..108: note = source = /note="Description of Artificial Sequence: Synthetic polynucleotide"
  source 1..108: mol_type = other RNA
gctggtgctgcagcttattatgtgggttaagtaggacttcgattggatggaataaaatataatgaaaatggaaccattacagatgctgtagactgtgcacttgaccct

SEQ ID NO: 5 - RNA, 82 nt, synthetic construct
  misc_feature 1..82: note = source = /note="Description of Artificial Sequence: Synthetic oligonucleotide"
  source 1..82: mol_type = other RNA
tctggttactgccagttgaatctgagggtccggacggatatcgcactaagtgtacctggtgcatttcgctgattttggggtc

SEQ ID NO: 6 - RNA, 82 nt, synthetic construct
  misc_feature 1..82: note = source = /note="Description of Artificial Sequence: Synthetic oligonucleotide"
  source 1..82: mol_type = other RNA
tctggttactgccagttgaatctgagggtcccatgaccatgtcactggctacactgaggtgcatttcgctgattttggggtc

SEQ ID NO: 7 - RNA, 82 nt, synthetic construct
  misc_feature 1..82: note = source = /note="Description of Artificial Sequence: Synthetic oligonucleotide"
  source 1..82: mol_type = other RNA
tctggttactgccagttgaatctgagggtccttgacatggcatgtgactccactgtcggtgcatttcgctgattttggggtc

SEQ ID NO: 8 - RNA, 82 nt, synthetic construct
  misc_feature 1..82: note = source = /note="Description of Artificial Sequence: Synthetic oligonucleotide"
  source 1..82: mol_type = other RNA
tctggttactgccagttgaatctgagggtccacctttgccagatgactgagtggaagggtgcatttcgctgattttggggtc

SEQ ID NO: 9 - RNA, 82 nt, synthetic construct
  misc_feature 1..82: note = source = /note="Description of Artificial Sequence: Synthetic oligonucleotide"
  source 1..82: mol_type = other RNA
tctggttactgccagttgaatctgagggtccagcttgaagcgttcgcgacaagtgtcggtgcatttcgctgattttggggtc

SEQ ID NO: 10 - RNA, 82 nt, synthetic construct
  misc_feature 1..82: note = source = /note="Description of Artificial Sequence: Synthetic oligonucleotide"
  source 1..82: mol_type = other RNA
tctggttactgccagttgaatctgagggtcctcacgtcctgagatcaactgctacatggtgcatttcgctgattttggggtc

SEQ ID NO: 11 - RNA, 82 nt, synthetic construct
  misc_feature 1..82: note = source = /note="Description of Artificial Sequence: Synthetic oligonucleotide"
  source 1..82: mol_type = other RNA
tctggttactgccagttgaatctgagggtccgttgactgatcacatgctgctccacgggtgcatttcgctgattttggggtc

SEQ ID NO: 12 - RNA, 82 nt, synthetic construct
  misc_feature 1..82: note = source = /note="Description of Artificial Sequence: Synthetic oligonucleotide"
  source 1..82: mol_type = other RNA
tctggttactgccagttgaatctgagggtcccagacagtcatcggattgatgagtgaggtgcatttcgctgattttggggtc

SEQ ID NO: 13 - DNA, 74 bp, synthetic construct
  misc_feature 1..74: note = source = /note="Description of Artificial Sequence: Synthetic oligonucleotide"
  source 1..74: mol_type = other DNA
taatacgactcactatagggctggtgctgcagcttattatgtgggtatagaacaacctaggacttttctattaa

SEQ ID NO: 14 - DNA, 26 bp, synthetic construct
  misc_feature 1..26: note = source = /note="Description of Artificial Sequence: Synthetic oligonucleotide"
  source 1..26: mol_type = other DNA
aacgtacactttgtttctgagagagg

SEQ ID NO: 15 - DNA, 37 bp, synthetic construct
  misc_feature 1..37: note = source = /note="Description of Artificial Sequence: Synthetic oligonucleotide"
  source 1..37: mol_type = other DNA
ctgacctgaaggctgacgccggacttgtggagacagc

SEQ ID NO: 16 - DNA, 59 bp, synthetic construct
  misc_feature 1..59: note = source = /note="Description of Artificial Sequence: Synthetic oligonucleotide"
  source 1..59: mol_type = other DNA
taatacgactcactatagggagatttggacctgcgagcgggttctgacctgaaggctga

SEQ ID NO: 17 - DNA, 39 bp, synthetic construct
  misc_feature 1..39: note = source = /note="Description of Artificial Sequence: Synthetic oligonucleotide"
  source 1..39: mol_type = other DNA
ggtttttcaatttcctgtttcttttccttaaagtcaacg

SEQ ID NO: 18 - DNA, 27 bp, synthetic construct
  misc_feature 1..27: note = source = /note="Description of Artificial Sequence: Synthetic primer"
  source 1..27: mol_type = other DNA
gctggtgctgcagcttattatgtgggt

SEQ ID NO: 19 - DNA, 20 bp, synthetic construct
  misc_feature 1..20: note = source = /note="Description of Artificial Sequence: Synthetic primer"
  source 1..20: mol_type = other DNA
agggtcaagtgcacagtcta

SEQ ID NO: 20 - DNA, 20 bp, synthetic construct
  misc_feature 1..20: note = source = /note="Description of Artificial Sequence: Synthetic primer"
  source 1..20: mol_type = other DNA
gaccccaaaatcagcgaaat

SEQ ID NO: 21 - DNA, 24 bp, synthetic construct
  misc_feature 1..24: note = source = /note="Description of Artificial Sequence: Synthetic primer"
  source 1..24: mol_type = other DNA
tctggttactgccagttgaatctg

SEQ ID NO: 22 - DNA, 53 bp, synthetic construct
  modified_base 25..34: mod_base = OTHER; note = a, c, t, g, unknown or other
  misc_feature 1..53: note = source = /note="Description of Artificial Sequence: Synthetic oligonucleotide"
  source 1..53: mol_type = other DNA
caagcagaagacggcatacgagatnnnnnnnnnnaccccaaaatcagcgaaat

SEQ ID NO: 23 - DNA, 63 bp, synthetic construct
  modified_base 30..39: mod_base = OTHER; note = a, c, t, g, unknown or other
  misc_feature 1..63: note = source = /note="Description of Artificial Sequence: Synthetic oligonucleotide"
  source 1..63: mol_type = other DNA
aatgatacggcgaccaccgagatctacacnnnnnnnnnntctggttactgccagttgaatctg

SEQ ID NO: 24 - DNA, 22 bp, synthetic construct
  misc_feature 1..22: note = source = /note="Description of Artificial Sequence: Synthetic primer"
  source 1..22: mol_type = other DNA
gaccaatcytgtcacctctgac

SEQ ID NO: 25 - DNA, 22 bp, synthetic construct
  misc_feature 1..22: note = source = /note="Description of Artificial Sequence: Synthetic primer"
  source 1..22: mol_type = other DNA
gaccaatyctgtcacctytgac

SEQ ID NO: 26 - DNA, 24 bp, synthetic construct
  misc_feature 1..24: note = source = /note="Description of Artificial Sequence: Synthetic primer"
  source 1..24: mol_type = other DNA
agggcattttggayaaagcgtcta

SEQ ID NO: 27 - DNA, 18 bp, synthetic construct
  misc_feature 1..18: note = source = /note="Description of Artificial Sequence: Synthetic primer"
  source 1..18: mol_type = other DNA
ttggggtcctcatcggag

SEQ ID NO: 28 - DNA, 21 bp, synthetic construct
  misc_feature 1..21: note = source = /note="Description of Artificial Sequence: Synthetic primer"
  source 1..21: mol_type = other DNA
ttctccaagcgaatctctgta

SEQ ID NO: 29 - DNA, 18 bp, synthetic construct
  misc_feature 1..18: note = source = /note="Description of Artificial Sequence: Synthetic primer"
  source 1..18: mol_type = other DNA
aagatggccatcggatcc

SEQ ID NO: 30 - DNA, 23 bp, synthetic construct
  misc_feature 1..23: note = source = /note="Description of Artificial Sequence: Synthetic primer"
  source 1..23: mol_type = other DNA
gtctccctcttctggtgataatc

SEQ ID NO: 31 - DNA, 106 bp, synthetic construct
  misc_feature 1..106: note = source = /note="Description of Artificial Sequence: Synthetic polynucleotide"
  source 1..106: mol_type = other DNA
gaccgatcctgtcacctctgactaagggtggcacaacgcagtgtgttgagctcccttagtagggtgactagcaccggcagcgtagacgctttgtccaaaatgccct

SEQ ID NO: 32 - DNA, 81 bp, synthetic construct
  misc_feature 1..81: note = source = /note="Description of Artificial Sequence: Synthetic oligonucleotide"
  source 1..81: mol_type = other DNA
ttggggtcctcatcggaggacgcttaaataatagtaggaacgttcgagtctctaaaaatatacagagattcgcttggagaa

SEQ ID NO: 33 - DNA, 140 bp, synthetic construct
  misc_feature 1..140: note = source = /note="Description of Artificial Sequence: Synthetic polynucleotide"
  source 1..140: mol_type = other DNA
aagatggccatcggatcctcaactcactcctgtaatgagtcgtagacaaggataagaggcccgatcggcagtatttcgccctttctaaaaataatgtgacctgggacgcactgcaccgattatcaccagaagagggagac

SEQ ID NO: 34-99 - skipped (66 entries)

SEQ ID NO: 100 - DNA, 25 bp, synthetic construct
  misc_feature 1..25: note = source = /note="Description of Artificial Sequence: Synthetic oligonucleotide"
  source 1..25: mol_type = other DNA
tggggtcttacacggcgatcttgcc

SEQ ID NO: 101 - DNA, 25 bp, synthetic construct
  misc_feature 1..25: note = source = /note="Description of Artificial Sequence: Synthetic oligonucleotide"
  source 1..25: mol_type = other DNA
gggtcaacgtgtcggcatggattct

SEQ ID NO: 102 - DNA, 28 bp, synthetic construct
  misc_feature 1..28: note = source = /note="Description of Artificial Sequence: Synthetic oligonucleotide"
  source 1..28: mol_type = other DNA
agttacattcacgccagttgtgtctggt

SEQ ID NO: 103 - DNA, 25 bp, synthetic construct
  misc_feature 1..25: note = source = /note="Description of Artificial Sequence: Synthetic oligonucleotide"
  source 1..25: mol_type = other DNA
agttacattcacgccagttgtggcg

SEQ ID NO: 104 - DNA, 26 bp, synthetic construct
  misc_feature 1..26: note = source = /note="Description of Artificial Sequence: Synthetic oligonucleotide"
  source 1..26: mol_type = other DNA
gtttgtaattacacggcgatcttgcc

SEQ ID NO: 105 - DNA, 28 bp, synthetic construct
  misc_feature 1..28: note = source = /note="Description of Artificial Sequence: Synthetic oligonucleotide"
  source 1..28: mol_type = other DNA
gtccaaatctttacacggcgatcttgcc

SEQ ID NO: 106 - DNA, 26 bp, synthetic construct
  misc_feature 1..26: note = source = /note="Description of Artificial Sequence: Synthetic oligonucleotide"
  source 1..26: mol_type = other DNA
agttacattcacgccagttgtggagc

SEQ ID NO: 107 - DNA, 43 bp, synthetic construct
  misc_feature 1..43: note = source = /note="Description of Artificial Sequence: Synthetic oligonucleotide"
  source 1..43: mol_type = other DNA
taatacgactcactatagggtctgataatggaccccaaaatca

SEQ ID NO: 108 - DNA, 21 bp, synthetic construct
  misc_feature 1..21: note = source = /note="Description of Artificial Sequence: Synthetic oligonucleotide"
  source 1..21: mol_type = other DNA
ttaggcctgagttgagtcagc

SEQ ID NO: 109 - DNA, 52 bp, synthetic construct
  misc_feature 1..52: note = source = /note="Description of Artificial Sequence: Synthetic oligonucleotide"
  source 1..52: mol_type = other DNA
caagcagaagacggcatacgagatgttctatcgaccccaaaatcagcgaaat

SEQ ID NO: 110 - DNA, 61 bp, synthetic construct
  misc_feature 1..61: note = source = /note="Description of Artificial Sequence: Synthetic oligonucleotide"
  source 1..61: mol_type = other DNA
aatgatacggcgaccaccgagatctacacaagatctgtctggttactgccagttgaatctg

SEQ ID NO: 111 - DNA, 52 bp, synthetic construct
  misc_feature 1..52: note = source = /note="Description of Artificial Sequence: Synthetic oligonucleotide"
  source 1..52: mol_type = other DNA
caagcagaagacggcatacgagatgttctatcttacaaacattggccgcaaa

SEQ ID NO: 112 - DNA, 55 bp, synthetic construct
  misc_feature 1..55: note = source = /note="Description of Artificial Sequence: Synthetic oligonucleotide"
  source 1..55: mol_type = other DNA
aatgatacggcgaccaccgagatctacacaagatctggcgcgacattccgaagaa

SEQ ID NO: 113 - DNA, 51 bp, synthetic construct
  misc_feature 1..51: note = source = /note="Description of Artificial Sequence: Synthetic oligonucleotide"
  source 1..51: mol_type = other DNA
caagcagaagacggcatacgagatgttctatcagatttggacctgcgagcg

SEQ ID NO: 114 - DNA, 57 bp, synthetic construct
  misc_feature 1..57: note = source = /note="Description of Artificial Sequence: Synthetic oligonucleotide"
  source 1..57: mol_type = other DNA
aatgatacggcgaccaccgagatctacacaagatctggagcggctgtctccacaagt

SEQ ID NO: 115 - DNA, 54 bp, synthetic construct
  misc_feature 1..54: note = source = /note="Description of Artificial Sequence: Synthetic oligonucleotide"
  source 1..54: mol_type = other DNA
caagcagaagacggcatacgagatgttctatctaatcagacaaggaactgatta

SEQ ID NO: 116 - DNA, 56 bp, synthetic construct
  misc_feature 1..56: note = source = /note="Description of Artificial Sequence: Synthetic oligonucleotide"
  source 1..56: mol_type = other DNA
aatgatacggcgaccaccgagatctacacaagatctgcgaaggtgtgacttccatg

SEQ ID NO: 117 - DNA, 57 bp, synthetic construct
  misc_feature 1..57: note = source = /note="Description of Artificial Sequence: Synthetic oligonucleotide"
  source 1..57: mol_type = other DNA
aatgatacggcgaccaccgagatctacacaagatctggatcaaaacaacgtcggccc

SEQ ID NO: 118 - DNA, 52 bp, synthetic construct
  misc_feature 1..52: note = source = /note="Description of Artificial Sequence: Synthetic oligonucleotide"
  source 1..52: mol_type = other DNA
caagcagaagacggcatacgagatgttctatcccatgttgagtgagagcggt

SEQ ID NO: 119 - DNA, 57 bp, synthetic construct
  misc_feature 1..57: note = source = /note="Description of Artificial Sequence: Synthetic oligonucleotide"
  source 1..57: mol_type = other DNA
aatgatacggcgaccaccgagatctacacaagatctgtggaccccaaaatcagcgaa

SEQ ID NO: 120 - DNA, 53 bp, synthetic construct
  misc_feature 1..53: note = source = /note="Description of Artificial Sequence: Synthetic oligonucleotide"
  source 1..53: mol_type = other DNA
caagcagaagacggcatacgagatgttctatcactgcgttctccattctggtt

SEQ ID NO: 121 - DNA, 57 bp, synthetic construct
  misc_feature 1..57: note = source = /note="Description of Artificial Sequence: Synthetic oligonucleotide"
  source 1..57: mol_type = other DNA
aatgatacggcgaccaccgagatctacacaagatctgcagcgttcttcggaatgtcg

SEQ ID NO: 122 - DNA, 52 bp, synthetic construct
  misc_feature 1..52: note = source = /note="Description of Artificial Sequence: Synthetic oligonucleotide"
  source 1..52: mol_type = other DNA
caagcagaagacggcatacgagatgttctatcgcacctgtgtaggtcaacca

SEQ ID NO: 123 - DNA, 57 bp, synthetic construct
  misc_feature 1..57: note = source = /note="Description of Artificial Sequence: Synthetic oligonucleotide"
  source 1..57: mol_type = other DNA
aatgatacggcgaccaccgagatctacacaagatctggaaatgcaccccgcattacg

SEQ ID NO: 124 - DNA, 52 bp, synthetic construct
  misc_feature 1..52: note = source = /note="Description of Artificial Sequence: Synthetic oligonucleotide"
  source 1..52: mol_type = other DNA
caagcagaagacggcatacgagatgttctatccccactgcgttctccattct

SEQ ID NO: 125 - DNA, 57 bp, synthetic construct
  misc_feature 1..57: note = source = /note="Description of Artificial Sequence: Synthetic oligonucleotide"
  source 1..57: mol_type = other DNA
aatgatacggcgaccaccgagatctacacaagatctggtcttggttcaccgctctca

SEQ ID NO: 126 - DNA, 51 bp, synthetic construct
  misc_feature 1..51: note = source = /note="Description of Artificial Sequence: Synthetic oligonucleotide"
  source 1..51: mol_type = other DNA
caagcagaagacggcatacgagatgttctatcttggaacgccttgtcctcg

SEQ ID NO: 127 - DNA, 57 bp, synthetic construct
  misc_feature 1..57: note = source = /note="Description of Artificial Sequence: Synthetic oligonucleotide"
  source 1..57: mol_type = other DNA
aatgatacggcgaccaccgagatctacacaagatctggcagtcaagcctcttctcgt

SEQ ID NO: 128 - DNA, 52 bp, synthetic construct
  misc_feature 1..52: note = source = /note="Description of Artificial Sequence: Synthetic oligonucleotide"
  source 1..52: mol_type = other DNA
caagcagaagacggcatacgagatgttctatcgaagttcccctactgctgcc

SEQ ID NO: 129 - DNA, 57 bp, synthetic construct
  misc_feature 1..57: note = source = /note="Description of Artificial Sequence: Synthetic oligonucleotide"
  source 1..57: mol_type = other DNA
aatgatacggcgaccaccgagatctacacaagatctgcgtttggtggaccctcagat

SEQ ID NO: 130 - DNA, 52 bp, synthetic construct
  misc_feature 1..52: note = source = /note="Description of Artificial Sequence: Synthetic oligonucleotide"
  source 1..52: mol_type = other DNA
caagcagaagacggcatacgagatgttctatcgacgttgttttgatcgcgcc

SEQ ID NO: 131 - DNA, 57 bp, synthetic construct
  misc_feature 1..57: note = source = /note="Description of Artificial Sequence: Synthetic oligonucleotide"
  source 1..57: mol_type = other DNA
aatgatacggcgaccaccgagatctacacaagatctgaaggccaacaacaacaaggc

SEQ ID NO: 132 - DNA, 52 bp, synthetic construct
  misc_feature 1..52: note = source = /note="Description of Artificial Sequence: Synthetic oligonucleotide"
  source 1..52: mol_type = other DNA
caagcagaagacggcatacgagatgttctatcggcagtacgtttttgccgag

SEQ ID NO: 133 - DNA, 57 bp, synthetic construct
  misc_feature 1..57: note = source = /note="Description of Artificial Sequence: Synthetic oligonucleotide"
  source 1..57: mol_type = other DNA
aatgatacggcgaccaccgagatctacacaagatctgaccagaatggagaacgcagt

SEQ ID NO: 134 - DNA, 52 bp, synthetic construct
  misc_feature 1..52: note = source = /note="Description of Artificial Sequence: Synthetic oligonucleotide"
  source 1..52: mol_type = other DNA
caagcagaagacggcatacgagatgttctatccggtgaaccaagacgcagta

SEQ ID NO: 135 - DNA, 57 bp, synthetic construct
  misc_feature 1..57: note = source = /note="Description of Artificial Sequence: Synthetic oligonucleotide"
  source 1..57: mol_type = other DNA
aatgatacggcgaccaccgagatctacacaagatctgccgcattacgtttggtggac

SEQ ID NO: 136 - DNA, 52 bp, synthetic construct
  misc_feature 1..52: note = source = /note="Description of Artificial Sequence: Synthetic oligonucleotide"
  source 1..52: mol_type = other DNA
caagcagaagacggcatacgagatgttctatcggccgacgttgttttgatcg

SEQ ID NO: 137 - DNA, 57 bp, synthetic construct
  misc_feature 1..57: note = source = /note="Description of Artificial Sequence: Synthetic oligonucleotide"
  source 1..57: mol_type = other DNA
aatgatacggcgaccaccgagatctacacaagatctggcctcggcaaaaacgtactg

SEQ ID NO: 138 - DNA, 52 bp, synthetic construct
  misc_feature 1..52: note = source = /note="Description of Artificial Sequence: Synthetic oligonucleotide"
  source 1..52: mol_type = other DNA
caagcagaagacggcatacgagatgttctatcttgttctggaccacgtctgc

SEQ ID NO: 139 - DNA, 57 bp, synthetic construct
  misc_feature 1..57: note = source = /note="Description of Artificial Sequence: Synthetic oligonucleotide"
  source 1..57: mol_type = other DNA
aatgatacggcgaccaccgagatctacacaagatctgaattccctcgaggacaaggc

SEQ ID NO: 140 - DNA, 52 bp, synthetic construct
  misc_feature 1..52: note = source = /note="Description of Artificial Sequence: Synthetic oligonucleotide"
  source 1..52: mol_type = other DNA
caagcagaagacggcatacgagatgttctatctcgtctggtagctcttcggt

SEQ ID NO: 141 - DNA, 57 bp, synthetic construct
  misc_feature 1..57: note = source = /note="Description of Artificial Sequence: Synthetic oligonucleotide"
  source 1..57: mol_type = other DNA
aatgatacggcgaccaccgagatctacacaagatctggcttcagcgttcttcggaat

SEQ ID NO: 142 - DNA, 52 bp, synthetic construct
  misc_feature 1..52: note = source = /note="Description of Artificial Sequence: Synthetic oligonucleotide"
  source 1..52: mol_type = other DNA
caagcagaagacggcatacgagatgttctatctggcacctgtgtaggtcaac

SEQ ID NO: 143 - DNA, 57 bp, synthetic construct
  misc_feature 1..57: note = source = /note="Description of Artificial Sequence: Synthetic oligonucleotide"
  source 1..57: mol_type = other DNA
aatgatacggcgaccaccgagatctacacaagatctgagaatagagctcgcaccgta

SEQ ID NO: 144 - DNA, 52 bp, synthetic construct
  misc_feature 1..52: note = source = /note="Description of Artificial Sequence: Synthetic oligonucleotide"
  source 1..52: mol_type = other DNA
caagcagaagacggcatacgagatgttctatcctcctctagtggcggctatt

SEQ ID NO: 145 - DNA, 57 bp, synthetic construct
  misc_feature 1..57: note = source = /note="Description of Artificial Sequence: Synthetic oligonucleotide"
  source 1..57: mol_type = other DNA
aatgatacggcgaccaccgagatctacacaagatctggctggtgctgcagcttatta

SEQ ID NO: 146 - DNA, 52 bp, synthetic construct
  misc_feature 1..52: note = source = /note="Description of Artificial Sequence: Synthetic oligonucleotide"
  source 1..52: mol_type = other DNA
caagcagaagacggcatacgagatgttctatcagggtcaagtgcacagtcta

SEQ ID NO: 147 - DNA, 59 bp, synthetic construct
  misc_feature 1..59: note = source = /note="Description of Artificial Sequence: Synthetic oligonucleotide"
  source 1..59: mol_type = other DNA
aatgatacggcgaccaccgagatctacacaagatctgttcggaagagacaggtacgtta

SEQ ID NO: 148 - DNA, 51 bp, synthetic construct
  misc_feature 1..51: note = source = /note="Description of Artificial Sequence: Synthetic oligonucleotide"
  source 1..51: mol_type = other DNA
caagcagaagacggcatacgagatgttctatcagcagtacgcacacaatcg

SEQ ID NO: 149 - DNA, 57 bp, synthetic construct
  misc_feature 1..57: note = source = /note="Description of Artificial Sequence: Synthetic oligonucleotide"
  source 1..57: mol_type = other DNA
aatgatacggcgaccaccgagatctacacaagatctgcaatgctgcaatcgtgctac

SEQ ID NO: 150 - DNA, 52 bp, synthetic construct
  misc_feature 1..52: note = source = /note="Description of Artificial Sequence: Synthetic oligonucleotide"
  source 1..52: mol_type = other DNA
caagcagaagacggcatacgagatgttctatcgttgcgactacgtgatgagg

SEQ ID NO: 151 - DNA, 19 bp, synthetic construct
  misc_feature 1..19: note = source = /note="Description of Artificial Sequence: Synthetic oligonucleotide"
  source 1..19: mol_type = other DNA
agatttggacctgcgagcg

SEQ ID NO: 152 - DNA, 20 bp, synthetic construct
  misc_feature 1..20: note = source = /note="Description of Artificial Sequence: Synthetic oligonucleotide"
  source 1..20: mol_type = other DNA
gagcggctgtctccacaagt

SEQ ID NO: 153 - DNA, 20 bp, synthetic construct
  misc_feature 1..20: note = source = /note="Description of Artificial Sequence: Synthetic oligonucleotide"
  source 1..20: mol_type = other DNA
agaatagagctcgcaccgta

SEQ ID NO: 154 - DNA, 20 bp, synthetic construct
  misc_feature 1..20: note = source = /note="Description of Artificial Sequence: Synthetic oligonucleotide"
  source 1..20: mol_type = other DNA
ctcctctagtggcggctatt

SEQ ID NO: 155 - DNA, 20 bp, synthetic construct
  misc_feature 1..20: note = source = /note="Description of Artificial Sequence: Synthetic oligonucleotide"
  source 1..20: mol_type = other DNA
gctggtgctgcagcttatta

SEQ ID NO: 156 - DNA, 20 bp, synthetic construct
  misc_feature 1..20: note = source = /note="Description of Artificial Sequence: Synthetic oligonucleotide"
  source 1..20: mol_type = other DNA
agggtcaagtgcacagtcta

SEQ ID NO: 157 - DNA, 22 bp, synthetic construct
  misc_feature 1..22: note = source = /note="Description of Artificial Sequence: Synthetic oligonucleotide"
  source 1..22: mol_type = other DNA
ttcggaagagacaggtacgtta

SEQ ID NO: 158 - DNA, 19 bp, synthetic construct
  misc_feature 1..19: note = source = /note="Description of Artificial Sequence: Synthetic oligonucleotide"
  source 1..19: mol_type = other DNA
agcagtacgcacacaatcg

SEQ ID NO: 159 - DNA, 20 bp, synthetic construct
  misc_feature 1..20: note = source = /note="Description of Artificial Sequence: Synthetic oligonucleotide"
  source 1..20: mol_type = other DNA
caatgctgcaatcgtgctac

SEQ ID NO: 160 - DNA, 20 bp, synthetic construct
  misc_feature 1..20: note = source = /note="Description of Artificial Sequence: Synthetic oligonucleotide"
  source 1..20: mol_type = other DNA
gttgcgactacgtgatgagg

SEQ ID NO: 161 - DNA, 20 bp, synthetic construct
  misc_feature 1..20: note = source = /note="Description of Artificial Sequence: Synthetic oligonucleotide"
  source 1..20: mol_type = other DNA
gaccccaaaatcagcgaaat

SEQ ID NO: 162 - DNA, 24 bp, synthetic construct
  misc_feature 1..24: note = source = /note="Description of Artificial Sequence: Synthetic oligonucleotide"
  source 1..24: mol_type = other DNA
tctggttactgccagttgaatctg

SEQ ID NO: 163 - DNA, 20 bp, synthetic construct
  misc_feature 1..20: note = source = /note="Description of Artificial Sequence: Synthetic oligonucleotide"
  source 1..20: mol_type = other DNA
ttacaaacattggccgcaaa

SEQ ID NO: 164 - DNA, 18 bp, synthetic construct
  misc_feature 1..18: note = source = /note="Description of Artificial Sequence: Synthetic oligonucleotide"
  source 1..18: mol_type = other DNA
gcgcgacattccgaagaa

SEQ ID NO: 165 - DNA, 22 bp, synthetic construct
  misc_feature 1..22: note = source = /note="Description of Artificial Sequence: Synthetic oligonucleotide"
  source 1..22: mol_type = other DNA
taatcagacaaggaactgatta

SEQ ID NO: 166 - DNA, 19 bp, synthetic construct
  misc_feature 1..19: note = source = /note="Description of Artificial Sequence: Synthetic oligonucleotide"
  source 1..19: mol_type = other DNA
cgaaggtgtgacttccatg

SEQ ID NO: 167 - DNA, 20 bp, synthetic construct
  misc_feature 1..20: note = source = /note="Description of Artificial Sequence: Synthetic oligonucleotide"
  source 1..20: mol_type = other DNA
gatcaaaacaacgtcggccc

SEQ ID NO: 168 - DNA, 20 bp, synthetic construct
  misc_feature 1..20: note = source = /note="Description of Artificial Sequence: Synthetic oligonucleotide"
  source 1..20: mol_type = other DNA
ccatgttgagtgagagcggt

SEQ ID NO: 169 - DNA, 20 bp, synthetic construct
  misc_feature 1..20: note = source = /note="Description of Artificial Sequence: Synthetic oligonucleotide"
  source 1..20: mol_type = other DNA
tggaccccaaaatcagcgaa

SEQ ID NO: 170 - DNA, 21 bp, synthetic construct
  misc_feature 1..21: note = source = /note="Description of Artificial Sequence: Synthetic oligonucleotide"
  source 1..21: mol_type = other DNA
actgcgttctccattctggtt

SEQ ID NO: 171 - DNA, 20 bp, synthetic construct
  misc_feature 1..20: note = source = /note="Description of Artificial Sequence: Synthetic oligonucleotide"
  source 1..20: mol_type = other DNA
cagcgttcttcggaatgtcg

SEQ ID NO: 172 - DNA, 20 bp, synthetic construct
  misc_feature 1..20: note = source = /note="Description of Artificial Sequence: Synthetic oligonucleotide"
  source 1..20: mol_type = other DNA
gcacctgtgtaggtcaacca

SEQ ID NO: 173 - DNA, 20 bp, synthetic construct
  misc_feature 1..20: note = source = /note="Description of Artificial Sequence: Synthetic oligonucleotide"
  source 1..20: mol_type = other DNA
gaaatgcaccccgcattacg

SEQ ID NO: 174 - DNA, 20 bp, synthetic construct
  misc_feature 1..20: note = source = /note="Description of Artificial Sequence: Synthetic oligonucleotide"
  source 1..20: mol_type = other DNA
cccactgcgttctccattct

SEQ ID NO: 175 - DNA, 20 bp, synthetic construct
  misc_feature 1..20: note = source = /note="Description of Artificial Sequence: Synthetic oligonucleotide"
  source 1..20: mol_type = other DNA
gtcttggttcaccgctctca

SEQ ID NO: 176 - DNA, 19 bp, synthetic construct
  misc_feature 1..19: note = source = /note="Description of Artificial Sequence: Synthetic oligonucleotide"
  source 1..19: mol_type = other DNA
ttggaacgccttgtcctcg

SEQ ID NO: 177 - DNA, 20 bp, synthetic construct
  misc_feature 1..20: note = source = /note="Description of Artificial Sequence: Synthetic oligonucleotide"
  source 1..20: mol_type = other DNA
gcagtcaagcctcttctcgt

SEQ ID NO: 178 - DNA, 20 bp, synthetic construct
  misc_feature 1..20: note = source = /note="Description of Artificial Sequence: Synthetic oligonucleotide"
  source 1..20: mol_type = other DNA
gaagttcccctactgctgcc

SEQ ID NO: 179 - DNA, 20 bp, synthetic construct
  misc_feature 1..20: note = source = /note="Description of Artificial Sequence: Synthetic oligonucleotide"
  source 1..20: mol_type = other DNA
cgtttggtggaccctcagat

SEQ ID NO: 180 - DNA, 20 bp, synthetic construct
  misc_feature 1..20: note = source = /note="Description of Artificial Sequence: Synthetic oligonucleotide"
  source 1..20: mol_type = other DNA
gacgttgttttgatcgcgcc

SEQ ID NO: 181 - DNA, 20 bp, synthetic construct
  misc_feature 1..20: note = source = /note="Description of Artificial Sequence: Synthetic oligonucleotide"
  source 1..20: mol_type = other DNA
aaggccaacaacaacaaggc

SEQ ID NO: 182 - DNA, 20 bp, synthetic construct
  misc_feature 1..20: note = source = /note="Description of Artificial Sequence: Synthetic oligonucleotide"
  source 1..20: mol_type = other DNA
ggcagtacgtttttgccgag

SEQ ID NO: 183 - DNA, 20 bp, synthetic construct
  misc_feature 1..20: note = source = /note="Description of Artificial Sequence: Synthetic oligonucleotide"
  source 1..20: mol_type = other DNA
accagaatggagaacgcagt

SEQ ID NO: 184 - DNA, 20 bp, synthetic construct
  misc_feature 1..20: note = source = /note="Description of Artificial Sequence: Synthetic oligonucleotide"
  source 1..20: mol_type = other DNA
cggtgaaccaagacgcagta

SEQ ID NO: 185 - DNA, 20 bp, synthetic construct
  misc_feature 1..20: note = source = /note="Description of Artificial Sequence: Synthetic oligonucleotide"
  source 1..20: mol_type = other DNA
ccgcattacgtttggtggac

SEQ ID NO: 186 - DNA, 20 bp, synthetic construct
  misc_feature 1..20: note = source = /note="Description of Artificial Sequence: Synthetic oligonucleotide"
  source 1..20: mol_type = other DNA
ggccgacgttgttttgatcg

SEQ ID NO: 187 - DNA, 20 bp, synthetic construct
  misc_feature 1..20: note = source = /note="Description of Artificial Sequence: Synthetic oligonucleotide"
  source 1..20: mol_type = other DNA
gcctcggcaaaaacgtactg

SEQ ID NO: 188 - DNA, 20 bp, synthetic construct
  misc_feature 1..20: note = source = /note="Description of Artificial Sequence: Synthetic oligonucleotide"
  source 1..20: mol_type = other DNA
ttgttctggaccacgtctgc

SEQ ID NO: 189 - DNA, 20 bp, synthetic construct
  misc_feature 1..20: note = source = /note="Description of Artificial Sequence: Synthetic oligonucleotide"
  source 1..20: mol_type = other DNA
aattccctcgaggacaaggc

SEQ ID NO: 190 - DNA, 20 bp, synthetic construct
  misc_feature 1..20: note = source = /note="Description of Artificial Sequence: Synthetic oligonucleotide"
  source 1..20: mol_type = other DNA
tcgtctggtagctcttcggt

SEQ ID NO: 191 - DNA, 20 bp, synthetic construct
  misc_feature 1..20: note = source = /note="Description of Artificial Sequence: Synthetic oligonucleotide"
  source 1..20: mol_type = other DNA
gcttcagcgttcttcggaat

SEQ ID NO: 192 - DNA, 20 bp, synthetic construct
  misc_feature 1..20: note = source = /note="Description of Artificial Sequence: Synthetic oligonucleotide"
  source 1..20: mol_type = other DNA
tggcacctgtgtaggtcaac

SEQ ID NO: 193 - DNA, 42 bp, synthetic construct
  misc_feature 1..42: note = source = /note="Description of Artificial Sequence: Synthetic oligonucleotide"
  source 1..42: mol_type = other DNA
gggtcacgcgtaggagttctatcagatttggacctgcgagcg

SEQ ID NO: 194 - DNA, 43 bp, synthetic construct
  misc_feature 1..43: note = source = /note="Description of Artificial Sequence: Synthetic oligonucleotide"
  source 1..43: mol_type = other DNA
gttccgcagccacacaagatctggagcggctgtctccacaagt

SEQ ID NO: 195 - DNA, 42 bp, synthetic construct
  misc_feature 1..42: note = source = /note="Description of Artificial Sequence: Synthetic oligonucleotide"
  source 1..42: mol_type = other DNA
cgcgtcgagtagggtgttctatcagatttggacctgcgagcg

SEQ ID NO: 196 - DNA, 43 bp, synthetic construct
  misc_feature 1..43: note = source = /note="Description of Artificial Sequence: Synthetic oligonucleotide"
  source 1..43: mol_type = other DNA
gccgtgtgaagctggaagatctggagcggctgtctccacaagt

SEQ ID NO: 197 - DNA, 42 bp, synthetic construct
  misc_feature 1..42: note = source = /note="Description of Artificial Sequence: Synthetic oligonucleotide"
  source 1..42: mol_type = other DNA
cgatcgcccttggtggttctatcagatttggacctgcgagcg

SEQ ID NO: 198 - DNA, 43 bp, synthetic construct
  misc_feature 1..43: note = source = /note="Description of Artificial Sequence: Synthetic oligonucleotide"
  source 1..43: mol_type = other DNA
ggtttagccggcgtgaagatctggagcggctgtctccacaagt

SEQ ID NO: 199 - DNA, 42 bp, synthetic construct
  misc_feature 1..42: note = source = /note="Description of Artificial Sequence: Synthetic oligonucleotide"
  source 1..42: mol_type = other DNA
ggtcgagccggaactgttctatcagatttggacctgcgagcg

SEQ ID NO: 200 - DNA, 43 bp, synthetic construct
  misc_feature 1..43: note = source = /note="Description of Artificial Sequence: Synthetic oligonucleotide"
  source 1..43: mol_type = other DNA
ggatgcgcacccagaaagatctggagcggctgtctccacaagt

SEQ ID NO: 201 - DNA, 42 bp, synthetic construct
  misc_feature 1..42: note = source = /note="Description of Artificial Sequence: Synthetic oligonucleotide"
  source 1..42: mol_type = other DNA
tcccggcgttgtcctgttctatcagatttggacctgcgagcg

SEQ ID NO: 202 - DNA, 43 bp, synthetic construct
  misc_feature 1..43: note = source = /note="Description of Artificial Sequence: Synthetic oligonucleotide"
  source 1..43: mol_type = other DNA
gctccgtcactgcccaagatctggagcggctgtctccacaagt

SEQ ID NO: 203 - DNA, 42 bp, synthetic construct
  misc_feature 1..42: note = source = /note="Description of Artificial Sequence: Synthetic oligonucleotide"
  source 1..42: mol_type = other DNA
cgcagggtccagagtgttctatcagatttggacctgcgagcg

SEQ ID NO: 204 - DNA, 43 bp, synthetic construct
  misc_feature 1..43: note = source = /note="Description of Artificial Sequence: Synthetic oligonucleotide"
  source 1..43: mol_type = other DNA
gttcgcgcgaaggaaaagatctggagcggctgtctccacaagt

SEQ ID NO: 205 - DNA, 47 bp, synthetic construct
  misc_feature 1..47: note = source = /note="Description of Artificial Sequence: Synthetic oligonucleotide"
  source 1..47: mol_type = other DNA
atatagatgccgtcctagcggttctatcagatttggacctgcgagcg

SEQ ID NO: 206 - DNA, 48 bp, synthetic construct
  misc_feature 1..48: note = source = /note="Description of Artificial Sequence: Synthetic oligonucleotide"
  source 1..48: mol_type = other DNA
aagtatctttcctgtgcccaaagatctggagcggctgtctccacaagt

SEQ ID NO: 207 - DNA, 47 bp, synthetic construct
  misc_feature 1..47: note = source = /note="Description of Artificial Sequence: Synthetic oligonucleotide"
  source 1..47: mol_type = other DNA
ccctttaatcagatgcgtcggttctatcagatttggacctgcgagcg

SEQ ID NO: 208 - DNA, 48 bp, synthetic construct
  misc_feature 1..48: note = source = /note="Description of Artificial Sequence: Synthetic oligonucleotide"
  source 1..48: mol_type = other DNA
tggtagtaataagggcgaccaagatctggagcggctgtctccacaagt

SEQ ID NO: 209 - DNA, 47 bp, synthetic construct
  misc_feature 1..47: note = source = /note="Description of Artificial Sequence: Synthetic oligonucleotide"
  source 1..47: mol_type = other DNA
ttggtcatgtgcttttcgttgttctatcagatttggacctgcgagcg

SEQ ID NO: 210 - DNA, 48 bp, synthetic construct
  misc_feature 1..48: note = source = /note="Description of Artificial Sequence: Synthetic oligonucleotide"
  source 1..48: mol_type = other DNA
aggggtatcggatactcagaaagatctggagcggctgtctccacaagt

SEQ ID NO: 211 - DNA, 47 bp, synthetic construct
  misc_feature 1..47: note = source = /note="Description of Artificial Sequence: Synthetic oligonucleotide"
  source 1..47: mol_type = other DNA
gggtgggtaaatggtaatgcgttctatcagatttggacctgcgagcg

SEQ ID NO: 212 - DNA, 48 bp, synthetic construct
  misc_feature 1..48: note = source = /note="Description of Artificial Sequence: Synthetic oligonucleotide"
  source 1..48: mol_type = other DNA
atcgattccccggatatagcaagatctggagcggctgtctccacaagt

SEQ ID NO: 213 - DNA, 47 bp, synthetic construct
  misc_feature 1..47: note = source = /note="Description of Artificial Sequence: Synthetic oligonucleotide"
  source 1..47: mol_type = other DNA
tccgacggggagtatatactgttctatcagatttggacctgcgagcg

SEQ ID NO: 214 - DNA, 48 bp, synthetic construct
  misc_feature 1..48: note = source = /note="Description of Artificial Sequence: Synthetic oligonucleotide"
  source 1..48: mol_type = other DNA
tactaactgcttcaggccaaaagatctggagcggctgtctccacaagt

SEQ ID NO: 215 - DNA, 47 bp, synthetic construct
  misc_feature 1..47: note = source = /note="Description of Artificial Sequence: Synthetic oligonucleotide"
  source 1..47: mol_type = other DNA
catgtttaggaacgctaccggttctatcagatttggacctgcgagcg

SEQ ID NO: 216 - DNA, 48 bp, synthetic construct
  misc_feature 1..48: note = source = /note="Description of Artificial Sequence: Synthetic oligonucleotide"
  source 1..48: mol_type = other DNA
aataatctccgttccctcccaagatctggagcggctgtctccacaagt

SEQ ID NO: 217 - DNA, 79 bp, synthetic construct
  misc_feature 1..79: note = source = /note="Description of Artificial Sequence: Synthetic oligonucleotide"
  source 1..79: mol_type = other DNA
taatacgactcactatagggaccccaaaatcagcgaaatgcaccccgcattacgaaaccaggaccctcagattcaactg

SEQ ID NO: 218 - DNA, 22 bp, synthetic construct
  misc_feature 1..22: note = source = /note="Description of Artificial Sequence: Synthetic oligonucleotide"
  source 1..22: mol_type = other DNA
cgcagtattattgggtaaacct

SEQ ID NO: 219 - DNA, 74 bp, synthetic construct; identical to SEQ ID NO: 13
  misc_feature 1..74: note = source = /note="Description of Artificial Sequence: Synthetic oligonucleotide"
  source 1..74: mol_type = other DNA

SEQ ID NO: 220 - DNA, 26 bp, synthetic construct
  misc_feature 1..26: note = source = /note="Description of Artificial Sequence: Synthetic oligonucleotide"
  source 1..26: mol_type = other DNA
aacgtacactttgtttctgagagagg

SEQ ID NO: 221 - DNA, 52 bp, synthetic construct
  misc_feature 1..52: note = source = /note="Description of Artificial Sequence: Synthetic oligonucleotide"
  source 1..52: mol_type = other DNA
caagcagaagacggcatacgagatgagtcttcgaccccaaaatcagcgaaat

SEQ ID NO: 222 - DNA, 52 bp, synthetic construct; identical to SEQ ID NO: 109
  misc_feature 1..52: note = source = /note="Description of Artificial Sequence: Synthetic oligonucleotide"
  source 1..52: mol_type = other DNA

SEQ ID NO: 223 - DNA, 52 bp, synthetic construct
  misc_feature 1..52: note = source = /note="Description of Artificial Sequence: Synthetic oligonucleotide"
  source 1..52: mol_type = other DNA
caagcagaagacggcatacgagattgggccaagaccccaaaatcagcgaaat

SEQ ID NO: 224 - DNA, 52 bp, synthetic construct
  misc_feature 1..52: note = source = /note="Description of Artificial Sequence: Synthetic oligonucleotide"
  source 1..52: mol_type = other DNA
caagcagaagacggcatacgagatattgttgggaccccaaaatcagcgaaat

SEQ ID NO: 225 - DNA, 52 bp, synthetic construct
  misc_feature 1..52: note = source = /note="Description of Artificial Sequence: Synthetic oligonucleotide"
  source 1..52: mol_type = other DNA
caagcagaagacggcatacgagattcccgttggaccccaaaatcagcgaaat

SEQ ID NO: 226 - DNA, 52 bp, synthetic construct
  misc_feature 1..52: note = source = /note="Description of Artificial Sequence: Synthetic oligonucleotide"
  source 1..52: mol_type = other DNA
caagcagaagacggcatacgagatacacacttgaccccaaaatcagcgaaat

SEQ ID NO: 227 - DNA, 52 bp, synthetic construct
  misc_feature 1..52: note = source = /note="Description of Artificial Sequence: Synthetic oligonucleotide"
  source 1..52: mol_type = other DNA
caagcagaagacggcatacgagatccattccagaccccaaaatcagcgaaat

SEQ ID NO: 228 - DNA, 52 bp, synthetic construct
  misc_feature 1..52: note = source = /note="Description of Artificial Sequence: Synthetic oligonucleotide"
  source 1..52: mol_type = other DNA
caagcagaagacggcatacgagatctaacggggaccccaaaatcagcgaaat

SEQ ID NO: 229 - DNA, 52 bp, synthetic construct
  misc_feature 1..52: note = source = /note="Description of Artificial Sequence: Synthetic oligonucleotide"
  source 1..52: mol_type = other DNA
caagcagaagacggcatacgagatccataggagaccccaaaatcagcgaaat

SEQ ID NO: 230 - DNA, 52 bp, synthetic construct
  misc_feature 1..52: note = source = /note="Description of Artificial Sequence: Synthetic oligonucleotide"
  source 1..52: mol_type = other DNA
caagcagaagacggcatacgagatcagtgtaggaccccaaaatcagcgaaat

SEQ ID NO: 231 - DNA, 52 bp, synthetic construct
  misc_feature 1..52: note = source = /note="Description of Artificial Sequence: Synthetic oligonucleotide"
  source 1..52: mol_type = other DNA
caagcagaagacggcatacgagatgattctcagaccccaaaatcagcgaaat

SEQ ID NO: 232 - DNA, 52 bp, synthetic construct
  misc_feature 1..52: note = source = /note="Description of Artificial Sequence: Synthetic oligonucleotide"
  source 1..52: mol_type = other DNA
caagcagaagacggcatacgagatccttcttagaccccaaaatcagcgaaat

SEQ ID NO: 233 - DNA, 52 bp, synthetic construct
  misc_feature 1..52: note = source = /note="Description of Artificial Sequence: Synthetic oligonucleotide"
  source 1..52: mol_type = other DNA
caagcagaagacggcatacgagattctaagacgaccccaaaatcagcgaaat

SEQ ID NO: 234 - DNA, 52 bp, synthetic construct
  misc_feature 1..52: note = source = /note="Description of Artificial Sequence: Synthetic oligonucleotide"
  source 1..52: mol_type = other DNA
caagcagaagacggcatacgagatgcggcatagaccccaaaatcagcgaaat

SEQ ID NO: 235 - DNA, 52 bp, synthetic construct
  misc_feature 1..52: note = source = /note="Description of Artificial Sequence: Synthetic oligonucleotide"
  source 1..52: mol_type = other DNA
caagcagaagacggcatacgagatattgacgagaccccaaaatcagcgaaat

SEQ ID NO: 236 - DNA, 52 bp, synthetic construct
  misc_feature 1..52: note = source = /note="Description of Artificial Sequence: Synthetic oligonucleotide"
  source 1..52: mol_type = other DNA
caagcagaagacggcatacgagatgctcctgagaccccaaaatcagcgaaat

SEQ ID NO: 237 - DNA, 52 bp, synthetic construct
  misc_feature 1..52: note = source = /note="Description of Artificial Sequence: Synthetic oligonucleotide"
  source 1..52: mol_type = other DNA
caagcagaagacggcatacgagatgcaatcctgaccccaaaatcagcgaaat

SEQ ID NO: 238 - DNA, 52 bp, synthetic construct
  misc_feature 1..52: note = source = /note="Description of Artificial Sequence: Synthetic oligonucleotide"
  source 1..52: mol_type = other DNA
caagcagaagacggcatacgagatatgtcgttgaccccaaaatcagcgaaat

SEQ ID NO: 239 - DNA, 52 bp, synthetic construct
  misc_feature 1..52: note = source = /note="Description of Artificial Sequence: Synthetic oligonucleotide"
  source 1..52: mol_type = other DNA
caagcagaagacggcatacgagatttctcggcgaccccaaaatcagcgaaat

SEQ ID NO: 240 - DNA, 52 bp, synthetic construct
  misc_feature 1..52: note = source = /note="Description of Artificial Sequence: Synthetic oligonucleotide"
  source 1..52: mol_type = other DNA
caagcagaagacggcatacgagatcagggctagaccccaaaatcagcgaaat

SEQ ID NO: 241 - DNA, 52 bp, synthetic construct
  misc_feature 1..52: note = source = /note="Description of Artificial Sequence: Synthetic oligonucleotide"
  source 1..52: mol_type = other DNA
caagcagaagacggcatacgagatagccaagcgaccccaaaatcagcgaaat

SEQ ID NO: 242 - DNA, 52 bp, synthetic construct
  misc_feature 1..52: note = source = /note="Description of Artificial Sequence: Synthetic oligonucleotide"
  source 1..52: mol_type = other DNA
caagcagaagacggcatacgagataagcctgagaccccaaaatcagcgaaat

SEQ ID NO: 243 - DNA, 52 bp, synthetic construct
  misc_feature 1..52: note = source = /note="Description of Artificial Sequence: Synthetic oligonucleotide"
  source 1..52: mol_type = other DNA
caagcagaagacggcatacgagatctacagaggaccccaaaatcagcgaaat

SEQ ID NO: 244 - DNA, 52 bp, synthetic construct
  misc_feature 1..52: note = source = /note="Description of Artificial Sequence: Synthetic oligonucleotide"
  source 1..52: mol_type = other DNA
caagcagaagacggcatacgagatcgtagtcggaccccaaaatcagcgaaat

SEQ ID NO: 245 - DNA, 52 bp, synthetic construct
  misc_feature 1..52: note = source = /note="Description of Artificial Sequence: Synthetic oligonucleotide"
  source 1..52: mol_type = other DNA
caagcagaagacggcatacgagatttctgctcgaccccaaaatcagcgaaat

SEQ ID NO: 246 - DNA, 52 bp, synthetic construct
  misc_feature 1..52: note = source = /note="Description of Artificial Sequence: Synthetic oligonucleotide"
  source 1..52: mol_type = other DNA
caagcagaagacggcatacgagatgtgcacacgaccccaaaatcagcgaaat

SEQ ID NO: 247 - DNA, 52 bp, synthetic construct
  misc_feature 1..52: note = source = /note="Description of Artificial Sequence: Synthetic oligonucleotide"
  source 1..52: mol_type = other DNA
caagcagaagacggcatacgagataaagctcagaccccaaaatcagcgaaat

SEQ ID NO: 248 - DNA, 52 bp, synthetic construct
  misc_feature 1..52: note = source = /note="Description of Artificial Sequence: Synthetic oligonucleotide"
  source 1..52: mol_type = other DNA
caagcagaagacggcatacgagatgacctcaggaccccaaaatcagcgaaat

SEQ ID NO: 249 - DNA, 52 bp, synthetic construct
  misc_feature 1..52: note = source = /note="Description of Artificial Sequence: Synthetic oligonucleotide"
  source 1..52: mol_type = other DNA
caagcagaagacggcatacgagatctttccaagaccccaaaatcagcgaaat

SEQ ID NO: 250 - DNA, 52 bp, synthetic construct
  misc_feature 1..52: note = source = /note="Description of Artificial Sequence: Synthetic oligonucleotide"
  source 1..52: mol_type = other DNA
caagcagaagacggcatacgagattcttggctgaccccaaaatcagcgaaat

SEQ ID NO: 251 - DNA, 52 bp, synthetic construct
  misc_feature 1..52: note = source = /note="Description of Artificial Sequence: Synthetic oligonucleotide"
  source 1..52: mol_type = other DNA
caagcagaagacggcatacgagatcgcgtctagaccccaaaatcagcgaaat

SEQ ID NO: 252 - DNA, 52 bp, synthetic construct
  misc_feature 1..52: note = source = /note="Description of Artificial Sequence: Synthetic oligonucleotide"
  source 1..52: mol_type = other DNA
caagcagaagacggcatacgagattcgcgctagaccccaaaatcagcgaaat

SEQ ID NO: 253 - DNA, 52 bp, synthetic construct
  misc_feature 1..52: note = source = /note="Description of Artificial Sequence: Synthetic oligonucleotide"
  source 1..52: mol_type = other DNA
caagcagaagacggcatacgagatatccattcgaccccaaaatcagcgaaat

SEQ ID NO: 254 - DNA, 52 bp, synthetic construct
  misc_feature 1..52: note = source = /note="Description of Artificial Sequence: Synthetic oligonucleotide"
  source 1..52: mol_type = other DNA
caagcagaagacggcatacgagatgcccagtagaccccaaaatcagcgaaat

SEQ ID NO: 255 - DNA, 52 bp, synthetic construct
  misc_feature 1..52: note = source = /note="Description of Artificial Sequence: Synthetic oligonucleotide"
  source 1..52: mol_type = other DNA
caagcagaagacggcatacgagattaccgacggaccccaaaatcagcgaaat

SEQ ID NO: 256 - DNA, 52 bp, synthetic construct
  misc_feature 1..52: note = source = /note="Description of Artificial Sequence: Synthetic oligonucleotide"
  source 1..52: mol_type = other DNA
caagcagaagacggcatacgagattccatacggaccccaaaatcagcgaaat

SEQ ID NO: 257 - DNA, 52 bp, synthetic construct
  misc_feature 1..52: note = source = /note="Description of Artificial Sequence: Synthetic oligonucleotide"
  source 1..52: mol_type = other DNA
caagcagaagacggcatacgagataacatgtcgaccccaaaatcagcgaaat

SEQ ID NO: 258 - DNA, 52 bp, synthetic construct
  misc_feature 1..52: note = source = /note="Description of Artificial Sequence: Synthetic oligonucleotide"
  source 1..52: mol_type = other DNA
caagcagaagacggcatacgagatcgactatagaccccaaaatcagcgaaat

SEQ ID NO: 259 - DNA, 52 bp, synthetic construct
  misc_feature 1..52: note = source = /note="Description of Artificial Sequence: Synthetic oligonucleotide"
  source 1..52: mol_type = other DNA
caagcagaagacggcatacgagatacccaaaggaccccaaaatcagcgaaat

SEQ ID NO: 260 - DNA, 52 bp, synthetic construct
  misc_feature 1..52: note = source = /note="Description of Artificial Sequence: Synthetic oligonucleotide"
  source 1..52: mol_type = other DNA
caagcagaagacggcatacgagatatcgatcggaccccaaaatcagcgaaat

SEQ ID NO: 261 - DNA, 52 bp, synthetic construct
  misc_feature 1..52: note = source = /note="Description of Artificial Sequence: Synthetic oligonucleotide"
  source 1..52: mol_type = other DNA
caagcagaagacggcatacgagatgttggatggaccccaaaatcagcgaaat

SEQ ID NO: 262 - DNA, 52 bp, synthetic construct
  misc_feature 1..52: note = source = /note="Description of Artificial Sequence: Synthetic oligonucleotide"
  source 1..52: mol_type = other DNA
caagcagaagacggcatacgagatctatgtgagaccccaaaatcagcgaaat

SEQ ID NO: 263 - DNA, 52 bp, synthetic construct
  misc_feature 1..52: note = source = /note="Description of Artificial Sequence: Synthetic oligonucleotide"
  source 1..52: mol_type = other DNA
caagcagaagacggcatacgagattatttcgcgaccccaaaatcagcgaaat

SEQ ID NO: 264 - DNA, 52 bp, synthetic construct
  misc_feature 1..52: note = source = /note="Description of Artificial Sequence: Synthetic oligonucleotide"
  source 1..52: mol_type = other DNA
caagcagaagacggcatacgagatccatgtatgaccccaaaatcagcgaaat

SEQ ID NO: 265 - DNA, 52 bp, synthetic construct
  misc_feature 1..52: note = source = /note="Description of Artificial Sequence: Synthetic oligonucleotide"
  source 1..52: mol_type = other DNA
caagcagaagacggcatacgagatgccacgttgaccccaaaatcagcgaaat

SEQ ID NO: 266 - DNA, 52 bp, synthetic construct
  misc_feature 1..52: note = source = /note="Description of Artificial Sequence: Synthetic oligonucleotide"
  source 1..52: mol_type = other DNA
caagcagaagacggcatacgagatgtcgtgtagaccccaaaatcagcgaaat

SEQ ID NO: 267 - DNA, 52 bp, synthetic construct
  misc_feature 1..52: note = source = /note="Description of Artificial Sequence: Synthetic oligonucleotide"
  source 1..52: mol_type = other DNA
caagcagaagacggcatacgagattaaagtcggaccccaaaatcagcgaaat

SEQ ID NO: 268 - DNA, 52 bp, synthetic construct
  misc_feature 1..52: note = source = /note="Description of Artificial Sequence: Synthetic oligonucleotide"
  source 1..52: mol_type = other DNA
caagcagaagacggcatacgagatcttcggacgaccccaaaatcagcgaaat

SEQ ID NO: 269 - DNA, 52 bp, synthetic construct
  misc_feature 1..52: note = source = /note="Description of Artificial Sequence: Synthetic oligonucleotide"
  source 1..52: mol_type = other DNA
caagcagaagacggcatacgagatgcactctcgaccccaaaatcagcgaaat

SEQ ID NO: 270 - DNA, 52 bp, synthetic construct
  misc_feature 1..52: note = source = /note="Description of Artificial Sequence: Synthetic oligonucleotide"
  source 1..52: mol_type = other DNA
caagcagaagacggcatacgagattcagatacgaccccaaaatcagcgaaat

SEQ ID NO: 271 - DNA, 52 bp, synthetic construct
  misc_feature 1..52: note = source = /note="Description of Artificial Sequence: Synthetic oligonucleotide"
  source 1..52: mol_type = other DNA
caagcagaagacggcatacgagatcagtccctgaccccaaaatcagcgaaat

SEQ ID NO: 272 - DNA, 52 bp, synthetic construct
  misc_feature 1..52: note = source = /note="Description of Artificial Sequence: Synthetic oligonucleotide"
  source 1..52: mol_type = other DNA
caagcagaagacggcatacgagatgccctaacgaccccaaaatcagcgaaat

SEQ ID NO: 273 - DNA, 52 bp, synthetic construct
  misc_feature 1..52: note = source = /note="Description of Artificial Sequence: Synthetic oligonucleotide"
  source 1..52: mol_type = other DNA
caagcagaagacggcatacgagatctgcatcagaccccaaaatcagcgaaat

SEQ ID NO: 274 - DNA, 52 bp, synthetic construct
  misc_feature 1..52: note = source = /note="Description of Artificial Sequence: Synthetic oligonucleotide"
  source 1..52: mol_type = other DNA
caagcagaagacggcatacgagatcggtatcggaccccaaaatcagcgaaat

SEQ ID NO: 275 - DNA, 52 bp, synthetic construct
  misc_feature 1..52: note = source = /note="Description of Artificial Sequence: Synthetic oligonucleotide"
  source 1..52: mol_type = other DNA
caagcagaagacggcatacgagataagtatgggaccccaaaatcagcgaaat

SEQ ID NO: 276 - DNA, 52 bp, synthetic construct
  misc_feature 1..52: note = source = /note="Description of Artificial Sequence: Synthetic oligonucleotide"
  source 1..52: mol_type = other DNA
caagcagaagacggcatacgagatattcgcgcgaccccaaaatcagcgaaat

SEQ ID NO: 277 - DNA, 52 bp, synthetic construct
  misc_feature 1..52: note = source = /note="Description of Artificial Sequence: Synthetic oligonucleotide"
  source 1..52: mol_type = other DNA
caagcagaagacggcatacgagatatcaaggtgaccccaaaatcagcgaaat

SEQ ID NO: 278 - DNA, 52 bp, synthetic construct
  misc_feature 1..52: note = source = /note="Description of Artificial Sequence: Synthetic oligonucleotide"
  source 1..52: mol_type = other DNA
caagcagaagacggcatacgagatttgtgcatgaccccaaaatcagcgaaat

SEQ ID NO: 279 - DNA, 52 bp, synthetic construct
  misc_feature 1..52: note = source = /note="Description of Artificial Sequence: Synthetic oligonucleotide"
  source 1..52: mol_type = other DNA
caagcagaagacggcatacgagatctgtgctggaccccaaaatcagcgaaat

SEQ ID NO: 280 - DNA, 52 bp, synthetic construct
  misc_feature 1..52: note = source = /note="Description of Artificial Sequence: Synthetic oligonucleotide"
  source 1..52: mol_type = other DNA
caagcagaagacggcatacgagatgtccgtaggaccccaaaatcagcgaaat

SEQ ID NO: 281 - DNA, 52 bp, synthetic construct
  misc_feature 1..52: note = source = /note="Description of Artificial Sequence: Synthetic oligonucleotide"
  source 1..52: mol_type = other DNA
caagcagaagacggcatacgagatgttcaagagaccccaaaatcagcgaaat

SEQ ID NO: 282 - DNA, 52 bp, synthetic construct
  misc_feature 1..52: note = source = /note="Description of Artificial Sequence: Synthetic oligonucleotide"
  source 1..52: mol_type = other DNA
caagcagaagacggcatacgagatcaccgttcgaccccaaaatcagcgaaat

SEQ ID NO: 283 - DNA, 52 bp, synthetic construct
  misc_feature 1..52: note = source = /note="Description of Artificial Sequence: Synthetic oligonucleotide"
  source 1..52: mol_type = other DNA
caagcagaagacggcatacgagatcgagttgagaccccaaaatcagcgaaat

SEQ ID NO: 284 - DNA, 52 bp, synthetic construct
  misc_feature 1..52: note = source = /note="Description of Artificial Sequence: Synthetic oligonucleotide"
  source 1..52: mol_type = other DNA
caagcagaagacggcatacgagatgagcacgagaccccaaaatcagcgaaat

SEQ ID NO: 285 - DNA, 52 bp, synthetic construct
  misc_feature 1..52: note = source = /note="Description of Artificial Sequence: Synthetic oligonucleotide"
  source 1..52: mol_type = other DNA
caagcagaagacggcatacgagatagttcgtggaccccaaaatcagcgaaat

SEQ ID NO: 286 - DNA, 52 bp, synthetic construct
  misc_feature 1..52: note = source = /note="Description of Artificial Sequence: Synthetic oligonucleotide"
  source 1..52: mol_type = other DNA
caagcagaagacggcatacgagatcatcaactgaccccaaaatcagcgaaat

SEQ ID NO: 287 - DNA, 52 bp, synthetic construct
  misc_feature 1..52: note = source = /note="Description of Artificial Sequence: Synthetic oligonucleotide"
  source 1..52: mol_type = other DNA
caagcagaagacggcatacgagatcgagatctgaccccaaaatcagcgaaat

SEQ ID NO: 288 - DNA, 52 bp, synthetic construct
  misc_feature 1..52: note = source = /note="Description of Artificial Sequence: Synthetic oligonucleotide"
  source 1..52: mol_type = other DNA
caagcagaagacggcatacgagattggccagagaccccaaaatcagcgaaat

SEQ ID NO: 289 - DNA, 52 bp, synthetic construct
  misc_feature 1..52: note = source = /note="Description of Artificial Sequence: Synthetic oligonucleotide"
  source 1..52: mol_type = other DNA
caagcagaagacggcatacgagatttcaccatgaccccaaaatcagcgaaat

SEQ ID NO: 290 - DNA, 52 bp, synthetic construct
  misc_feature 1..52: note = source = /note="Description of Artificial Sequence: Synthetic oligonucleotide"
  source 1..52: mol_type = other DNA
caagcagaagacggcatacgagatgaatgcatgaccccaaaatcagcgaaat

SEQ ID NO: 291 - DNA, 52 bp, synthetic construct
  misc_feature 1..52: note = source = /note="Description of Artificial Sequence: Synthetic oligonucleotide"
  source 1..52: mol_type = other DNA
caagcagaagacggcatacgagattggaccctgaccccaaaatcagcgaaat

SEQ ID NO: 292 - DNA, 52 bp, synthetic construct
  misc_feature 1..52: note = source = /note="Description of Artificial Sequence: Synthetic oligonucleotide"
  source 1..52: mol_type = other DNA
caagcagaagacggcatacgagatgatagcacgaccccaaaatcagcgaaat

SEQ ID NO: 293 - DNA, 52 bp, synthetic construct
  misc_feature 1..52: note = source = /note="Description of Artificial Sequence: Synthetic oligonucleotide"
  source 1..52: mol_type = other DNA
caagcagaagacggcatacgagatacgacgacgaccccaaaatcagcgaaat

SEQ ID NO: 294 - DNA, 52 bp, synthetic construct
  misc_feature 1..52: note = source = /note="Description of Artificial Sequence: Synthetic oligonucleotide"
  source 1..52: mol_type = other DNA
caagcagaagacggcatacgagatctcagtatgaccccaaaatcagcgaaat

SEQ ID NO: 295 - DNA, 52 bp, synthetic construct
  misc_feature 1..52: note = source = /note="Description of Artificial Sequence: Synthetic oligonucleotide"
  source 1..52: mol_type = other DNA
caagcagaagacggcatacgagatcttagctagaccccaaaatcagcgaaat

SEQ ID NO: 296 - DNA, 52 bp, synthetic construct
  misc_feature 1..52: note = source = /note="Description of Artificial Sequence: Synthetic oligonucleotide"
  source 1..52: mol_type = other DNA
caagcagaagacggcatacgagatctgtttacgaccccaaaatcagcgaaat

SEQ ID NO: 297 - DNA, 52 bp, synthetic construct
  misc_feature 1..52: note = source = /note="Description of Artificial Sequence: Synthetic oligonucleotide"
  source 1..52: mol_type = other DNA
caagcagaagacggcatacgagattgtcccacgaccccaaaatcagcgaaat

SEQ ID NO: 298 - DNA, 52 bp, synthetic construct
  misc_feature 1..52: note = source = /note="Description of Artificial Sequence: Synthetic oligonucleotide"
  source 1..52: mol_type = other DNA
caagcagaagacggcatacgagattcctgagggaccccaaaatcagcgaaat

SEQ ID NO: 299 - DNA, 52 bp, synthetic construct
  misc_feature 1..52: note = source = /note="Description of Artificial Sequence: Synthetic oligonucleotide"
  source 1..52: mol_type = other DNA
caagcagaagacggcatacgagattagttccagaccccaaaatcagcgaaat

SEQ ID NO: 300 - DNA, 52 bp, synthetic construct
  misc_feature 1..52: note = source = /note="Description of Artificial Sequence: Synthetic oligonucleotide"
  source 1..52: mol_type = other DNA
caagcagaagacggcatacgagatcatgactcgaccccaaaatcagcgaaat

SEQ ID NO: 301 - DNA, 52 bp, synthetic construct
  misc_feature 1..52: note = source = /note="Description of Artificial Sequence: Synthetic oligonucleotide"
  source 1..52: mol_type = other DNA
caagcagaagacggcatacgagatgtaagcgcgaccccaaaatcagcgaaat

SEQ ID NO: 302 - DNA, 52 bp, synthetic construct
  misc_feature 1..52: note = source = /note="Description of Artificial Sequence: Synthetic oligonucleotide"
  source 1..52: mol_type = other DNA
caagcagaagacggcatacgagataacccagtgaccccaaaatcagcgaaat

SEQ ID NO: 303 - DNA, 52 bp, synthetic construct
  misc_feature 1..52: note = source = /note="Description of Artificial Sequence: Synthetic oligonucleotide"
  source 1..52: mol_type = other DNA
caagcagaagacggcatacgagattttgaggggaccccaaaatcagcgaaat

SEQ ID NO: 304 - DNA, 52 bp, synthetic construct
  misc_feature 1..52: note = source = /note="Description of Artificial Sequence: Synthetic oligonucleotide"
  source 1..52: mol_type = other DNA
caagcagaagacggcatacgagatagccgacagaccccaaaatcagcgaaat

SEQ ID NO: 305 - DNA, 52 bp, synthetic construct
  misc_feature 1..52: note = source = /note="Description of Artificial Sequence: Synthetic oligonucleotide"
  source 1..52: mol_type = other DNA
caagcagaagacggcatacgagataaacccgcgaccccaaaatcagcgaaat

SEQ ID NO: 306 - DNA, 52 bp, synthetic construct
  misc_feature 1..52: note = source = /note="Description of Artificial Sequence: Synthetic oligonucleotide"
  source 1..52: mol_type = other DNA
caagcagaagacggcatacgagatgtagggctgaccccaaaatcagcgaaat

SEQ ID NO: 307 - DNA, 52 bp, synthetic construct
  misc_feature 1..52: note = source = /note="Description of Artificial Sequence: Synthetic oligonucleotide"
  source 1..52: mol_type = other DNA
caagcagaagacggcatacgagatagacgattgaccccaaaatcagcgaaat

SEQ ID NO: 308 - DNA, 52 bp, synthetic construct
  misc_feature 1..52: note = source = /note="Description of Artificial Sequence: Synthetic oligonucleotide"
  source 1..52: mol_type = other DNA
caagcagaagacggcatacgagataggatgatgaccccaaaatcagcgaaat

SEQ ID NO: 309 - DNA, 52 bp, synthetic construct
  misc_feature 1..52: note = source = /note="Description of Artificial Sequence: Synthetic oligonucleotide"
  source 1..52: mol_type = other DNA
caagcagaagacggcatacgagatataatggcgaccccaaaatcagcgaaat

SEQ ID NO: 310 - DNA, 52 bp, synthetic construct
  misc_feature 1..52: note = source = /note="Description of Artificial Sequence: Synthetic oligonucleotide"
  source 1..52: mol_type = other DNA
caagcagaagacggcatacgagatcttggcgtgaccccaaaatcagcgaaat

SEQ ID NO: 311 - DNA, 52 bp, synthetic construct
  misc_feature 1..52: note = source = /note="Description of Artificial Sequence: Synthetic oligonucleotide"
  source 1..52: mol_type = other DNA
caagcagaagacggcatacgagatagctgtgcgaccccaaaatcagcgaaat

SEQ ID NO: 312 - DNA, 52 bp, synthetic construct
  misc_feature 1..52: note = source = /note="Description of Artificial Sequence: Synthetic oligonucleotide"
  source 1..52: mol_type = other DNA
caagcagaagacggcatacgagatgagtccaagaccccaaaatcagcgaaat

SEQ ID NO: 313 - DNA, 52 bp, synthetic construct
  misc_feature 1..52: note = source = /note="Description of Artificial Sequence: Synthetic oligonucleotide"
  source 1..52: mol_type = other DNA
caagcagaagacggcatacgagatgaataccagaccccaaaatcagcgaaat

SEQ ID NO: 314 - DNA, 52 bp, synthetic construct
  misc_feature 1..52: note = source = /note="Description of Artificial Sequence: Synthetic oligonucleotide"
  source 1..52: mol_type = other DNA
caagcagaagacggcatacgagataggagcttgaccccaaaatcagcgaaat

SEQ ID NO: 315 - DNA, 52 bp, synthetic construct
  misc_feature 1..52: note = source = /note="Description of Artificial Sequence: Synthetic oligonucleotide"
  source 1..52: mol_type = other DNA
caagcagaagacggcatacgagatgtgacttagaccccaaaatcagcgaaat

SEQ ID NO: 316 - DNA, 52 bp, synthetic construct
  misc_feature 1..52: note = source = /note="Description of Artificial Sequence: Synthetic oligonucleotide"
  source 1..52: mol_type = other DNA
caagcagaagacggcatacgagattttggaacgaccccaaaatcagcgaaat

SEQ ID NO: 317 - DNA, 52 bp, synthetic construct
  misc_feature 1..52: note = source = /note="Description of Artificial Sequence: Synthetic oligonucleotide"
  source 1..52: mol_type = other DNA
caagcagaagacggcatacgagatgagtcttcagggtcaagtgcacagtcta

SEQ ID NO: 318 - DNA, 52 bp, synthetic construct; identical to SEQ ID NO: 146
  misc_feature 1..52: note = source = /note="Description of Artificial Sequence: Synthetic oligonucleotide"
  source 1..52: mol_type = other DNA

SEQ ID NO: 319 - DNA, 52 bp, synthetic construct
  misc_feature 1..52: note = source = /note="Description of Artificial Sequence: Synthetic oligonucleotide"
  source 1..52: mol_type = other DNA
caagcagaagacggcatacgagattgggccaaagggtcaagtgcacagtcta

SEQ ID NO: 320 - DNA, 52 bp, synthetic construct
  misc_feature 1..52: note = source = /note="Description of Artificial Sequence: Synthetic oligonucleotide"
  source 1..52: mol_type = other DNA
caagcagaagacggcatacgagatattgttggagggtcaagtgcacagtcta

SEQ ID NO: 321 - DNA, 52 bp, synthetic construct
  misc_feature 1..52: note = source = /note="Description of Artificial Sequence: Synthetic oligonucleotide"
  source 1..52: mol_type = other DNA
caagcagaagacggcatacgagattcccgttgagggtcaagtgcacagtcta

SEQ ID NO: 322 - DNA, 52 bp, synthetic construct
  misc_feature 1..52: note = source = /note="Description of Artificial Sequence: Synthetic oligonucleotide"
  source 1..52: mol_type = other DNA
caagcagaagacggcatacgagatacacacttagggtcaagtgcacagtcta

SEQ ID NO: 323 - DNA, 52 bp, synthetic construct
  misc_feature 1..52: note = source = /note="Description of Artificial Sequence: Synthetic oligonucleotide"
  source 1..52: mol_type = other DNA
caagcagaagacggcatacgagatccattccaagggtcaagtgcacagtcta

SEQ ID NO: 324 - DNA, 52 bp, synthetic construct
  misc_feature 1..52: note = source = /note="Description of Artificial Sequence: Synthetic oligonucleotide"
  source 1..52: mol_type = other DNA
caagcagaagacggcatacgagatctaacgggagggtcaagtgcacagtcta

SEQ ID NO: 325 - DNA, 52 bp, synthetic construct
  misc_feature 1..52: note = source = /note="Description of Artificial Sequence: Synthetic oligonucleotide"
  source 1..52: mol_type = other DNA
caagcagaagacggcatacgagatccataggaagggtcaagtgcacagtcta

SEQ ID NO: 326 - DNA, 52 bp, synthetic construct
  misc_feature 1..52: note = source = /note="Description of Artificial Sequence: Synthetic oligonucleotide"
  source 1..52: mol_type = other DNA
caagcagaagacggcatacgagatcagtgtagagggtcaagtgcacagtcta

SEQ ID NO: 327 - DNA, 52 bp, synthetic construct
  misc_feature 1..52: note = source = /note="Description of Artificial Sequence: Synthetic oligonucleotide"
  source 1..52: mol_type = other DNA
caagcagaagacggcatacgagatgattctcaagggtcaagtgcacagtcta

SEQ ID NO: 328 - DNA, 52 bp, synthetic construct
  misc_feature 1..52: note = source = /note="Description of Artificial Sequence: Synthetic oligonucleotide"
  source 1..52: mol_type = other DNA
caagcagaagacggcatacgagatccttcttaagggtcaagtgcacagtcta

SEQ ID NO: 329 - DNA, 52 bp, synthetic construct
  misc_feature 1..52: note = source = /note="Description of Artificial Sequence: Synthetic oligonucleotide"
  source 1..52: mol_type = other DNA
caagcagaagacggcatacgagattctaagacagggtcaagtgcacagtcta

SEQ ID NO: 330 - DNA, 52 bp, synthetic construct
  misc_feature 1..52: note = source = /note="Description of Artificial Sequence: Synthetic oligonucleotide"
  source 1..52: mol_type = other DNA
caagcagaagacggcatacgagatgcggcataagggtcaagtgcacagtcta

SEQ ID NO: 331 - DNA, 52 bp, synthetic construct
  misc_feature 1..52: note = source = /note="Description of Artificial Sequence: Synthetic oligonucleotide"
  source 1..52: mol_type = other DNA
caagcagaagacggcatacgagatattgacgaagggtcaagtgcacagtcta

SEQ ID NO: 332 - DNA, 52 bp, synthetic construct
  misc_feature 1..52: note = source = /note="Description of Artificial Sequence: Synthetic oligonucleotide"
  source 1..52: mol_type = other DNA
caagcagaagacggcatacgagatgctcctgaagggtcaagtgcacagtcta

SEQ ID NO: 333 - DNA, 52 bp, synthetic construct
  misc_feature 1..52: note = source = /note="Description of Artificial Sequence: Synthetic oligonucleotide"
  source 1..52: mol_type = other DNA
caagcagaagacggcatacgagatgcaatcctagggtcaagtgcacagtcta

SEQ ID NO: 334 - DNA, 52 bp, synthetic construct
  misc_feature 1..52: note = source = /note="Description of Artificial Sequence: Synthetic oligonucleotide"
  source 1..52: mol_type = other DNA
caagcagaagacggcatacgagatatgtcgttagggtcaagtgcacagtcta

SEQ ID NO: 335 - DNA, 52 bp, synthetic construct
  misc_feature 1..52: note = source = /note="Description of Artificial Sequence: Synthetic oligonucleotide"
  source 1..52: mol_type = other DNA
caagcagaagacggcatacgagatttctcggcagggtcaagtgcacagtcta

SEQ ID NO: 336 - DNA, 52 bp, synthetic construct
  misc_feature 1..52: note = source = /note="Description of Artificial Sequence: Synthetic oligonucleotide"
  source 1..52: mol_type = other DNA
caagcagaagacggcatacgagatcagggctaagggtcaagtgcacagtcta

SEQ ID NO: 337 - DNA, 52 bp, synthetic construct
  misc_feature 1..52: note = source = /note="Description of Artificial Sequence: Synthetic oligonucleotide"
  source 1..52: mol_type = other DNA
caagcagaagacggcatacgagatagccaagcagggtcaagtgcacagtcta

SEQ ID NO: 338 - DNA, 52 bp, synthetic construct
  misc_feature 1..52: note = source = /note="Description of Artificial Sequence: Synthetic oligonucleotide"
  source 1..52: mol_type = other DNA
caagcagaagacggcatacgagataagcctgaagggtcaagtgcacagtcta

SEQ ID NO: 339 - DNA, 52 bp, synthetic construct
  misc_feature 1..52: note = source = /note="Description of Artificial Sequence: Synthetic oligonucleotide"
  source 1..52: mol_type = other DNA
caagcagaagacggcatacgagatctacagagagggtcaagtgcacagtcta

SEQ ID NO: 340 - DNA, 52 bp, synthetic construct
  misc_feature 1..52: note = source = /note="Description of Artificial Sequence: Synthetic oligonucleotide"
  source 1..52: mol_type = other DNA
caagcagaagacggcatacgagatcgtagtcgagggtcaagtgcacagtcta

SEQ ID NO: 341 - DNA, 52 bp, synthetic construct
  misc_feature 1..52: note = source = /note="Description of Artificial Sequence: Synthetic oligonucleotide"
  source 1..52: mol_type = other DNA
caagcagaagacggcatacgagatttctgctcagggtcaagtgcacagtcta

SEQ ID NO: 342 - DNA, 52 bp, synthetic construct
  misc_feature 1..52: note = source = /note="Description of Artificial Sequence: Synthetic oligonucleotide"
  source 1..52: mol_type = other DNA
caagcagaagacggcatacgagatgtgcacacagggtcaagtgcacagtcta

SEQ ID NO: 343 - DNA, 52 bp, synthetic construct
  misc_feature 1..52: note = source = /note="Description of Artificial Sequence: Synthetic oligonucleotide"
  source 1..52: mol_type = other DNA
caagcagaagacggcatacgagataaagctcaagggtcaagtgcacagtcta

SEQ ID NO: 344 - DNA, 52 bp, synthetic construct
  misc_feature 1..52: note = source = /note="Description of Artificial Sequence: Synthetic oligonucleotide"
  source 1..52: mol_type = other DNA
caagcagaagacggcatacgagatgacctcagagggtcaagtgcacagtcta

SEQ ID NO: 345 - DNA, 52 bp, synthetic construct
  misc_feature 1..52: note = source = /note="Description of Artificial Sequence: Synthetic oligonucleotide"
  source 1..52: mol_type = other DNA
caagcagaagacggcatacgagatctttccaaagggtcaagtgcacagtcta

SEQ ID NO: 346 - DNA, 52 bp, synthetic construct
  misc_feature 1..52: note = source = /note="Description of Artificial Sequence: Synthetic oligonucleotide"
  source 1..52: mol_type = other DNA
caagcagaagacggcatacgagattcttggctagggtcaagtgcacagtcta

SEQ ID NO: 347 - DNA, 52 bp, synthetic construct
  misc_feature 1..52: note = source = /note="Description of Artificial Sequence: Synthetic oligonucleotide"
  source 1..52: mol_type = other DNA
caagcagaagacggcatacgagatcgcgtctaagggtcaagtgcacagtcta

SEQ ID NO: 348 - DNA, 52 bp, synthetic construct
  misc_feature 1..52: note = source = /note="Description of Artificial Sequence: Synthetic oligonucleotide"
  source 1..52: mol_type = other DNA
caagcagaagacggcatacgagattcgcgctaagggtcaagtgcacagtcta

SEQ ID NO: 349 - DNA, 52 bp, synthetic construct
  misc_feature 1..52: note = source = /note="Description of Artificial Sequence: Synthetic oligonucleotide"
  source 1..52: mol_type = other DNA
caagcagaagacggcatacgagatatccattcagggtcaagtgcacagtcta

SEQ ID NO: 350 - DNA, 52 bp, synthetic construct
  misc_feature 1..52: note = source = /note="Description of Artificial Sequence: Synthetic oligonucleotide"
  source 1..52: mol_type = other DNA
caagcagaagacggcatacgagatgcccagtaagggtcaagtgcacagtcta

SEQ ID NO: 351 - DNA, 52 bp, synthetic construct
  misc_feature 1..52: note = source = /note="Description of Artificial Sequence: Synthetic oligonucleotide"
  source 1..52: mol_type = other DNA
caagcagaagacggcatacgagattaccgacgagggtcaagtgcacagtcta

SEQ ID NO: 352 - DNA, 52 bp, synthetic construct
  misc_feature 1..52: note = source = /note="Description of Artificial Sequence: Synthetic oligonucleotide"
  source 1..52: mol_type = other DNA
caagcagaagacggcatacgagattccatacgagggtcaagtgcacagtcta

SEQ ID NO: 353 - DNA, 52 bp, synthetic construct
  misc_feature 1..52: note = source = /note="Description of Artificial Sequence: Synthetic oligonucleotide"
  source 1..52: mol_type = other DNA
caagcagaagacggcatacgagataacatgtcagggtcaagtgcacagtcta

SEQ ID NO: 354 - DNA, 52 bp, synthetic construct
  misc_feature 1..52: note = source = /note="Description of Artificial Sequence: Synthetic oligonucleotide"
  source 1..52: mol_type = other DNA
caagcagaagacggcatacgagatcgactataagggtcaagtgcacagtcta

SEQ ID NO: 355 - DNA, 52 bp, synthetic construct
  misc_feature 1..52: note = source = /note="Description of Artificial Sequence: Synthetic oligonucleotide"
  source 1..52: mol_type = other DNA
caagcagaagacggcatacgagatacccaaagagggtcaagtgcacagtcta

SEQ ID NO: 356 - DNA, 52 bp, synthetic construct
  misc_feature 1..52: note = source = /note="Description of Artificial Sequence: Synthetic oligonucleotide"
  source 1..52: mol_type = other DNA
caagcagaagacggcatacgagatatcgatcgagggtcaagtgcacagtcta

SEQ ID NO: 357 - DNA, 52 bp, synthetic construct
  misc_feature 1..52: note = source = /note="Description of Artificial Sequence: Synthetic oligonucleotide"
  source 1..52: mol_type = other DNA
caagcagaagacggcatacgagatgttggatgagggtcaagtgcacagtcta

SEQ ID NO: 358 - DNA, 52 bp, synthetic construct
  misc_feature 1..52: note = source = /note="Description of Artificial Sequence: Synthetic oligonucleotide"
  source 1..52: mol_type = other DNA
caagcagaagacggcatacgagatctatgtgaagggtcaagtgcacagtcta

SEQ ID NO: 359 - DNA, 52 bp, synthetic construct
  misc_feature 1..52: note = source = /note="Description of Artificial Sequence: Synthetic oligonucleotide"
  source 1..52: mol_type = other DNA
caagcagaagacggcatacgagattatttcgcagggtcaagtgcacagtcta

SEQ ID NO: 360 - DNA, 52 bp, synthetic construct
  misc_feature 1..52: note = source = /note="Description of Artificial Sequence: Synthetic oligonucleotide"
  source 1..52: mol_type = other DNA
caagcagaagacggcatacgagatccatgtatagggtcaagtgcacagtcta

SEQ ID NO: 361 - DNA, 52 bp, synthetic construct
  misc_feature 1..52: note = source = /note="Description of Artificial Sequence: Synthetic oligonucleotide"
  source 1..52: mol_type = other DNA
caagcagaagacggcatacgagatgccacgttagggtcaagtgcacagtcta

SEQ ID NO: 362 - DNA, 52 bp, synthetic construct
  misc_feature 1..52: note = source = /note="Description of Artificial Sequence: Synthetic oligonucleotide"
  source 1..52: mol_type = other DNA
caagcagaagacggcatacgagatgtcgtgtaagggtcaagtgcacagtcta

SEQ ID NO: 363 - DNA, 52 bp, synthetic construct
  misc_feature 1..52: note = source = /note="Description of Artificial Sequence: Synthetic oligonucleotide"
  source 1..52: mol_type = other DNA
caagcagaagacggcatacgagattaaagtcgagggtcaagtgcacagtcta

SEQ ID NO: 364 - DNA, 52 bp, synthetic construct
  misc_feature 1..52: note = source = /note="Description of Artificial Sequence: Synthetic oligonucleotide"
  source 1..52: mol_type = other DNA
caagcagaagacggcatacgagatcttcggacagggtcaagtgcacagtcta

SEQ ID NO: 365 - DNA, 52 bp, synthetic construct
  misc_feature 1..52: note = source = /note="Description of Artificial Sequence: Synthetic oligonucleotide"
  source 1..52: mol_type = other DNA
caagcagaagacggcatacgagatgcactctcagggtcaagtgcacagtcta

SEQ ID NO: 366 - DNA, 52 bp, synthetic construct
  misc_feature 1..52: note = source = /note="Description of Artificial Sequence: Synthetic oligonucleotide"
  source 1..52: mol_type = other DNA
caagcagaagacggcatacgagattcagatacagggtcaagtgcacagtcta

SEQ ID NO: 367 - DNA, 52 bp, synthetic construct
  misc_feature 1..52: note = source = /note="Description of Artificial Sequence: Synthetic oligonucleotide"
  source 1..52: mol_type = other DNA
caagcagaagacggcatacgagatcagtccctagggtcaagtgcacagtcta

SEQ ID NO: 368 - DNA, 52 bp, synthetic construct
  misc_feature 1..52: note = source = /note="Description of Artificial Sequence: Synthetic oligonucleotide"
  source 1..52: mol_type = other DNA
caagcagaagacggcatacgagatgccctaacagggtcaagtgcacagtcta

SEQ ID NO: 369 - DNA, 52 bp, synthetic construct
  misc_feature 1..52: note = source = /note="Description of Artificial Sequence: Synthetic oligonucleotide"
  source 1..52: mol_type = other DNA
caagcagaagacggcatacgagatctgcatcaagggtcaagtgcacagtcta

SEQ ID NO: 370 - DNA, 52 bp, synthetic construct
  misc_feature 1..52: note = source = /note="Description of Artificial Sequence: Synthetic oligonucleotide"
  source 1..52: mol_type = other DNA
caagcagaagacggcatacgagatcggtatcgagggtcaagtgcacagtcta

SEQ ID NO: 371 - DNA, 52 bp, synthetic construct
  misc_feature 1..52: note = source = /note="Description of Artificial Sequence: Synthetic oligonucleotide"
  source 1..52: mol_type = other DNA
caagcagaagacggcatacgagataagtatggagggtcaagtgcacagtcta

SEQ ID NO: 372 - DNA, 52 bp, synthetic construct
  misc_feature 1..52: note = source = /note="Description of Artificial Sequence: Synthetic oligonucleotide"
  source 1..52: mol_type = other DNA
caagcagaagacggcatacgagatattcgcgcagggtcaagtgcacagtcta

SEQ ID NO: 373 - DNA, 52 bp, synthetic construct
  misc_feature 1..52: note = source = /note="Description of Artificial Sequence: Synthetic oligonucleotide"
  source 1..52: mol_type = other DNA
caagcagaagacggcatacgagatatcaaggtagggtcaagtgcacagtcta

SEQ ID NO: 374 - DNA, 52 bp, synthetic construct
  misc_feature 1..52: note = source = /note="Description of Artificial Sequence: Synthetic oligonucleotide"
  source 1..52: mol_type = other DNA
caagcagaagacggcatacgagatttgtgcatagggtcaagtgcacagtcta

SEQ ID NO: 375 - DNA, 52 bp, synthetic construct
  misc_feature 1..52: note = source = /note="Description of Artificial Sequence: Synthetic oligonucleotide"
  source 1..52: mol_type = other DNA
caagcagaagacggcatacgagatctgtgctgagggtcaagtgcacagtcta

SEQ ID NO: 376 - DNA, 52 bp, synthetic construct
  misc_feature 1..52: note = source = /note="Description of Artificial Sequence: Synthetic oligonucleotide"
  source 1..52: mol_type = other DNA
caagcagaagacggcatacgagatgtccgtagagggtcaagtgcacagtcta

SEQ ID NO: 377 - DNA, 52 bp, synthetic construct
  misc_feature 1..52: note = source = /note="Description of Artificial Sequence: Synthetic oligonucleotide"
  source 1..52: mol_type = other DNA
caagcagaagacggcatacgagatgttcaagaagggtcaagtgcacagtcta

SEQ ID NO: 378 - DNA, 52 bp, synthetic construct
  misc_feature 1..52: note = source = /note="Description of Artificial Sequence: Synthetic oligonucleotide"
  source 1..52: mol_type = other DNA
caagcagaagacggcatacgagatcaccgttcagggtcaagtgcacagtcta

SEQ ID NO: 379 - DNA, 52 bp, synthetic construct
  misc_feature 1..52: note = source = /note="Description of Artificial Sequence: Synthetic oligonucleotide"
  source 1..52: mol_type = other DNA
caagcagaagacggcatacgagatcgagttgaagggtcaagtgcacagtcta

SEQ ID NO: 380 - DNA, 52 bp, synthetic construct
  misc_feature 1..52: note = source = /note="Description of Artificial Sequence: Synthetic oligonucleotide"
  source 1..52: mol_type = other DNA
caagcagaagacggcatacgagatgagcacgaagggtcaagtgcacagtcta

SEQ ID NO: 381 - DNA, 52 bp, synthetic construct
  misc_feature 1..52: note = source = /note="Description of Artificial Sequence: Synthetic oligonucleotide"
  source 1..52: mol_type = other DNA
caagcagaagacggcatacgagatagttcgtgagggtcaagtgcacagtcta

SEQ ID NO: 382 - DNA, 52 bp, synthetic construct
  misc_feature 1..52: note = source = /note="Description of Artificial Sequence: Synthetic oligonucleotide"
  source 1..52: mol_type = other DNA
caagcagaagacggcatacgagatcatcaactagggtcaagtgcacagtcta

SEQ ID NO: 383 - DNA, 52 bp, synthetic construct
  misc_feature 1..52: note = source = /note="Description of Artificial Sequence: Synthetic oligonucleotide"
  source 1..52: mol_type = other DNA
caagcagaagacggcatacgagatcgagatctagggtcaagtgcacagtcta

SEQ ID NO: 384 - DNA, 52 bp, synthetic construct
  misc_feature 1..52: note = source = /note="Description of Artificial Sequence: Synthetic oligonucleotide"
  source 1..52: mol_type = other DNA
caagcagaagacggcatacgagattggccagaagggtcaagtgcacagtcta

SEQ ID NO: 385 - DNA, 52 bp, synthetic construct
  misc_feature 1..52: note = source = /note="Description of Artificial Sequence: Synthetic oligonucleotide"
  source 1..52: mol_type = other DNA
caagcagaagacggcatacgagatttcaccatagggtcaagtgcacagtcta

SEQ ID NO: 386 - DNA, 52 bp, synthetic construct
  misc_feature 1..52: note = source = /note="Description of Artificial Sequence: Synthetic oligonucleotide"
  source 1..52: mol_type = other DNA
caagcagaagacggcatacgagatgaatgcatagggtcaagtgcacagtcta

SEQ ID NO: 387 - DNA, 52 bp, synthetic construct
  misc_feature 1..52: note = source = /note="Description of Artificial Sequence: Synthetic oligonucleotide"
  source 1..52: mol_type = other DNA
caagcagaagacggcatacgagattggaccctagggtcaagtgcacagtcta

SEQ ID NO: 388 - DNA, 52 bp, synthetic construct
  misc_feature 1..52: note = source = /note="Description of Artificial Sequence: Synthetic oligonucleotide"
  source 1..52: mol_type = other DNA
caagcagaagacggcatacgagatgatagcacagggtcaagtgcacagtcta

SEQ ID NO: 389 - DNA, 52 bp, synthetic construct
  misc_feature 1..52: note = source = /note="Description of Artificial Sequence: Synthetic oligonucleotide"
  source 1..52: mol_type = other DNA
caagcagaagacggcatacgagatacgacgacagggtcaagtgcacagtcta

SEQ ID NO: 390 - DNA, 52 bp, synthetic construct
  misc_feature 1..52: note = source = /note="Description of Artificial Sequence: Synthetic oligonucleotide"
  source 1..52: mol_type = other DNA
caagcagaagacggcatacgagatctcagtatagggtcaagtgcacagtcta

SEQ ID NO: 391 - DNA, 52 bp, synthetic construct
  misc_feature 1..52: note = source = /note="Description of Artificial Sequence: Synthetic oligonucleotide"
  source 1..52: mol_type = other DNA
caagcagaagacggcatacgagatcttagctaagggtcaagtgcacagtcta

SEQ ID NO: 392 - DNA, 52 bp, synthetic construct
  misc_feature 1..52: note = source = /note="Description of Artificial Sequence: Synthetic oligonucleotide"
  source 1..52: mol_type = other DNA
caagcagaagacggcatacgagatctgtttacagggtcaagtgcacagtcta

SEQ ID NO: 393 - DNA, 52 bp, synthetic construct
  misc_feature 1..52: note = source = /note="Description of Artificial Sequence: Synthetic oligonucleotide"
  source 1..52: mol_type = other DNA
caagcagaagacggcatacgagattgtcccacagggtcaagtgcacagtcta

SEQ ID NO: 394 - DNA, 52 bp, synthetic construct
  misc_feature 1..52: note = source = /note="Description of Artificial Sequence: Synthetic oligonucleotide"
  source 1..52: mol_type = other DNA
caagcagaagacggcatacgagattcctgaggagggtcaagtgcacagtcta

SEQ ID NO: 395 - DNA, 52 bp, synthetic construct
  misc_feature 1..52: note = source = /note="Description of Artificial Sequence: Synthetic oligonucleotide"
  source 1..52: mol_type = other DNA
caagcagaagacggcatacgagattagttccaagggtcaagtgcacagtcta

SEQ ID NO: 396 - DNA, 52 bp, synthetic construct
  misc_feature 1..52: note = source = /note="Description of Artificial Sequence: Synthetic oligonucleotide"
  source 1..52: mol_type = other DNA
caagcagaagacggcatacgagatcatgactcagggtcaagtgcacagtcta

SEQ ID NO: 397 - DNA, 52 bp, synthetic construct
  misc_feature 1..52: note = source = /note="Description of Artificial Sequence: Synthetic oligonucleotide"
  source 1..52: mol_type = other DNA
caagcagaagacggcatacgagatgtaagcgcagggtcaagtgcacagtcta

SEQ ID NO: 398 - DNA, 52 bp, synthetic construct
  misc_feature 1..52: note = source = /note="Description of Artificial Sequence: Synthetic oligonucleotide"
  source 1..52: mol_type = other DNA
caagcagaagacggcatacgagataacccagtagggtcaagtgcacagtcta

SEQ ID NO: 399 - DNA, 52 bp, synthetic construct
  misc_feature 1..52: note = source = /note="Description of Artificial Sequence: Synthetic oligonucleotide"
  source 1..52: mol_type = other DNA
caagcagaagacggcatacgagattttgagggagggtcaagtgcacagtcta

SEQ ID NO: 400 - DNA, 52 bp, synthetic construct
  misc_feature 1..52: note = source = /note="Description of Artificial Sequence: Synthetic oligonucleotide"
  source 1..52: mol_type = other DNA
caagcagaagacggcatacgagatagccgacaagggtcaagtgcacagtcta

SEQ ID NO: 401 - DNA, 52 bp, synthetic construct
  misc_feature 1..52: note = source = /note="Description of Artificial Sequence: Synthetic oligonucleotide"
  source 1..52: mol_type = other DNA
caagcagaagacggcatacgagataaacccgcagggtcaagtgcacagtcta

SEQ ID NO: 402 - DNA, 52 bp, synthetic construct
  misc_feature 1..52: note = source = /note="Description of Artificial Sequence: Synthetic oligonucleotide"
  source 1..52: mol_type = other DNA
caagcagaagacggcatacgagatgtagggctagggtcaagtgcacagtcta

SEQ ID NO: 403 - DNA, 52 bp, synthetic construct
  misc_feature 1..52: note = source = /note="Description of Artificial Sequence: Synthetic oligonucleotide"
  source 1..52: mol_type = other DNA
caagcagaagacggcatacgagatagacgattagggtcaagtgcacagtcta

SEQ ID NO: 404 - DNA, 52 bp, synthetic construct
  misc_feature 1..52: note = source = /note="Description of Artificial Sequence: Synthetic oligonucleotide"
  source 1..52: mol_type = other DNA
caagcagaagacggcatacgagataggatgatagggtcaagtgcacagtcta

SEQ ID NO: 405 - DNA, 52 bp, synthetic construct
  misc_feature 1..52: note = source = /note="Description of Artificial Sequence: Synthetic oligonucleotide"
  source 1..52: mol_type = other DNA
caagcagaagacggcatacgagatataatggcagggtcaagtgcacagtcta

SEQ ID NO: 406 - DNA, 52 bp, synthetic construct
  misc_feature 1..52: note = source = /note="Description of Artificial Sequence: Synthetic oligonucleotide"
  source 1..52: mol_type = other DNA
caagcagaagacggcatacgagatcttggcgtagggtcaagtgcacagtcta

SEQ ID NO: 407 - DNA, 52 bp, synthetic construct
  misc_feature 1..52: note = source = /note="Description of Artificial Sequence: Synthetic oligonucleotide"
  source 1..52: mol_type = other DNA
caagcagaagacggcatacgagatagctgtgcagggtcaagtgcacagtcta

SEQ ID NO: 408 - DNA, 52 bp, synthetic construct
  misc_feature 1..52: note = source = /note="Description of Artificial Sequence: Synthetic oligonucleotide"
  source 1..52: mol_type = other DNA
caagcagaagacggcatacgagatgagtccaaagggtcaagtgcacagtcta

SEQ ID NO: 409 - DNA, 52 bp, synthetic construct
  misc_feature 1..52: note = source = /note="Description of Artificial Sequence: Synthetic oligonucleotide"
  source 1..52: mol_type = other DNA
caagcagaagacggcatacgagatgaataccaagggtcaagtgcacagtcta

SEQ ID NO: 410 - DNA, 52 bp, synthetic construct
  misc_feature 1..52: note = source = /note="Description of Artificial Sequence: Synthetic oligonucleotide"
  source 1..52: mol_type = other DNA
caagcagaagacggcatacgagataggagcttagggtcaagtgcacagtcta

SEQ ID NO: 411 - DNA, 52 bp, synthetic construct
  misc_feature 1..52: note = source = /note="Description of Artificial Sequence: Synthetic oligonucleotide"
  source 1..52: mol_type = other DNA
caagcagaagacggcatacgagatgtgacttaagggtcaagtgcacagtcta

SEQ ID NO: 412 - DNA, 52 bp, synthetic construct
  misc_feature 1..52: note = source = /note="Description of Artificial Sequence: Synthetic oligonucleotide"
  source 1..52: mol_type = other DNA
caagcagaagacggcatacgagattttggaacagggtcaagtgcacagtcta

SEQ ID NO: 413 - DNA, 61 bp, synthetic construct; identical to SEQ ID NO: 110
  misc_feature 1..61: note = source = /note="Description of Artificial Sequence: Synthetic oligonucleotide"
  source 1..61: mol_type = other DNA

SEQ ID NO: 414 - DNA, 61 bp, synthetic construct
  misc_feature 1..61: note = source = /note="Description of Artificial Sequence: Synthetic oligonucleotide"
  source 1..61: mol_type = other DNA
aatgatacggcgaccaccgagatctacactgtcatgatctggttactgccagttgaatctg

SEQ ID NO: 415 - DNA, 61 bp, synthetic construct
  misc_feature 1..61: note = source = /note="Description of Artificial Sequence: Synthetic oligonucleotide"
  source 1..61: mol_type = other DNA
aatgatacggcgaccaccgagatctacactgtaacagtctggttactgccagttgaatctg

SEQ ID NO: 416 - DNA, 61 bp, synthetic construct
  misc_feature 1..61: note = source = /note="Description of Artificial Sequence: Synthetic oligonucleotide"
  source 1..61: mol_type = other DNA
aatgatacggcgaccaccgagatctacacgcgcaacttctggttactgccagttgaatctg

SEQ ID NO: 417 - DNA, 52 bp, synthetic construct
  misc_feature 1..52: note = source = /note="Description of Artificial Sequence: Synthetic oligonucleotide"
  source 1..52: mol_type = other DNA
aatgatacggcgaccaccgatcgatggctctggttactgccagttgaatctg

SEQ ID NO: 418 - DNA, 52 bp, synthetic construct
  misc_feature 1..52: note = source = /note="Description of Artificial Sequence: Synthetic oligonucleotide"
  source 1..52: mol_type = other DNA
aatgatacggcgaccaccgacatggttttctggttactgccagttgaatctg

SEQ ID NO: 419 - DNA, 52 bp, synthetic construct
  misc_feature 1..52: note = source = /note="Description of Artificial Sequence: Synthetic oligonucleotide"
  source 1..52: mol_type = other DNA
aatgatacggcgaccaccgaacgaaagctctggttactgccagttgaatctg

SEQ ID NO: 420 - DNA, 52 bp, synthetic construct
  misc_feature 1..52: note = source = /note="Description of Artificial Sequence: Synthetic oligonucleotide"
  source 1..52: mol_type = other DNA
aatgatacggcgaccaccgagctctgattctggttactgccagttgaatctg

SEQ ID NO: 421 - DNA, 57 bp, synthetic construct
  misc_feature 1..57: note = source = /note="Description of Artificial Sequence: Synthetic oligonucleotide"
  source 1..57: mol_type = other DNA
aatgatacggcgaccaccgagatctacacatgccctcgctggtgctgcagcttatta

SEQ ID NO: 422 - DNA, 57 bp, synthetic construct
  misc_feature 1..57: note = source = /note="Description of Artificial Sequence: Synthetic oligonucleotide"
  source 1..57: mol_type = other DNA
aatgatacggcgaccaccgagatctacacctcagatggctggtgctgcagcttatta

SEQ ID NO: 423 - DNA, 57 bp, synthetic construct
  misc_feature 1..57: note = source = /note="Description of Artificial Sequence: Synthetic oligonucleotide"
  source 1..57: mol_type = other DNA
aatgatacggcgaccaccgagatctacacgtaatctggctggtgctgcagcttatta

SEQ ID NO: 424 - DNA, 57 bp, synthetic construct
  misc_feature 1..57: note = source = /note="Description of Artificial Sequence: Synthetic oligonucleotide"
  source 1..57: mol_type = other DNA
aatgatacggcgaccaccgagatctacacgcaagattgctggtgctgcagcttatta

SEQ ID NO: 425 - DNA, 48 bp, synthetic construct
  misc_feature 1..48: note = source = /note="Description of Artificial Sequence: Synthetic oligonucleotide"
  source 1..48: mol_type = other DNA
aatgatacggcgaccaccgaatacgccagctggtgctgcagcttatta

SEQ ID NO: 426 - DNA, 48 bp, synthetic construct
  misc_feature 1..48: note = source = /note="Description of Artificial Sequence: Synthetic oligonucleotide"
  source 1..48: mol_type = other DNA
aatgatacggcgaccaccgaaccagtcggctggtgctgcagcttatta

SEQ ID NO: 427 - DNA, 48 bp, synthetic construct
  misc_feature 1..48: note = source = /note="Description of Artificial Sequence: Synthetic oligonucleotide"
  source 1..48: mol_type = other DNA
aatgatacggcgaccaccgaaacacggagctggtgctgcagcttatta

SEQ ID NO: 428 - DNA, 48 bp, synthetic construct
  misc_feature 1..48: note = source = /note="Description of Artificial Sequence: Synthetic oligonucleotide"
  source 1..48: mol_type = other DNA
aatgatacggcgaccaccgactgcctaggctggtgctgcagcttatta

SEQ ID NO: 429 - DNA, 31 bp, synthetic construct
  misc_feature 1..31: note = source = /note="Description of Artificial Sequence: Synthetic oligonucleotide"
  source 1..31: mol_type = other DNA
tctggttactgccagttgaatctgagggtcc

SEQ ID NO: 430 - DNA, 25 bp, synthetic construct
  misc_feature 1..25: note = source = /note="Description of Artificial Sequence: Synthetic oligonucleotide"
  source 1..25: mol_type = other DNA
ggtgcatttcgctgattttggggtc

SEQ ID NO: 431 - DNA, 31 bp, synthetic construct
  misc_feature 1..31: note = source = /note="Description of Artificial Sequence: Synthetic oligonucleotide"
  source 1..31: mol_type = other DNA
ggaccctcagattcaactggcagtaaccaga

SEQ ID NO: 432 - DNA, 27 bp, synthetic construct
  misc_feature 1..27: note = source = /note="Description of Artificial Sequence: Synthetic oligonucleotide"
  source 1..27: mol_type = other DNA
gctggtgctgcagcttattatgtgggt

SEQ ID NO: 433 - DNA, 28 bp, synthetic construct
  misc_feature 1..28: note = source = /note="Description of Artificial Sequence: Synthetic oligonucleotide"
  source 1..28: mol_type = other DNA
agatgctgtagactgtgcacttgaccct

SEQ ID NO: 434 - DNA, 27 bp, synthetic construct
  misc_feature 1..27: note = source = /note="Description of Artificial Sequence: Synthetic oligonucleotide"
  source 1..27: mol_type = other DNA
acccacataataagctgcagcaccagc

SEQ ID NO: 435 - DNA, 23 bp, synthetic construct
  misc_feature 1..23: note = source = /note="Description of Artificial Sequence: Synthetic oligonucleotide"
  source 1..23: mol_type = other DNA
gagcggctgtctccacaagtccg

SEQ ID NO: 436 - DNA, 23 bp, synthetic construct
  misc_feature 1..23: note = source = /note="Description of Artificial Sequence: Synthetic oligonucleotide"
  source 1..23: mol_type = other DNA
acccgctcgcaggtccaaatctg

SEQ ID NO: 437 - DNA, 23 bp, synthetic construct
  misc_feature 1..23: note = source = /note="Description of Artificial Sequence: Synthetic oligonucleotide"
  source 1..23: mol_type = other DNA
cggacttgtggagacagccgctc

SEQ ID NO: 438 - DNA, 51 bp, synthetic construct
  misc_feature 1..51: note = source = /note="Description of Artificial Sequence: Synthetic oligonucleotide"
  source 1..51: mol_type = other DNA
caagcagaagacggcatacgagatgagtcttcagatttggacctgcgagcg

SEQ ID NO: 439 - DNA, 51 bp, synthetic construct; identical to SEQ ID NO: 113
  misc_feature 1..51: note = source = /note="Description of Artificial Sequence: Synthetic oligonucleotide"
  source 1..51: mol_type = other DNA

SEQ ID NO: 440 - DNA, 51 bp, synthetic construct
  misc_feature 1..51: note = source = /note="Description of Artificial Sequence: Synthetic oligonucleotide"
  source 1..51: mol_type = other DNA
caagcagaagacggcatacgagattgggccaaagatttggacctgcgagcg

SEQ ID NO: 441 - DNA, 51 bp, synthetic construct
  misc_feature 1..51: note = source = /note="Description of Artificial Sequence: Synthetic oligonucleotide"
  source 1..51: mol_type = other DNA
caagcagaagacggcatacgagatattgttggagatttggacctgcgagcg

SEQ ID NO: 442 - DNA, 51 bp, synthetic construct
  misc_feature 1..51: note = source = /note="Description of Artificial Sequence: Synthetic oligonucleotide"
  source 1..51: mol_type = other DNA
caagcagaagacggcatacgagattcccgttgagatttggacctgcgagcg

SEQ ID NO: 443 - DNA, 51 bp, synthetic construct
  misc_feature 1..51: note = source = /note="Description of Artificial Sequence: Synthetic oligonucleotide"
  source 1..51: mol_type = other DNA
caagcagaagacggcatacgagatacacacttagatttggacctgcgagcg

SEQ ID NO: 444 - DNA, 51 bp, synthetic construct
  misc_feature 1..51: note = source = /note="Description of Artificial Sequence: Synthetic oligonucleotide"
  source 1..51: mol_type = other DNA
caagcagaagacggcatacgagatccattccaagatttggacctgcgagcg

SEQ ID NO: 445 - DNA, 51 bp, synthetic construct
  misc_feature 1..51: note = source = /note="Description of Artificial Sequence: Synthetic oligonucleotide"
  source 1..51: mol_type = other DNA
caagcagaagacggcatacgagatctaacgggagatttggacctgcgagcg

SEQ ID NO: 446 - DNA, 51 bp, synthetic construct
  misc_feature 1..51: note = source = /note="Description of Artificial Sequence: Synthetic oligonucleotide"
  source 1..51: mol_type = other DNA
caagcagaagacggcatacgagatccataggaagatttggacctgcgagcg

SEQ ID NO: 447 - DNA, 51 bp, synthetic construct
  misc_feature 1..51: note = source = /note="Description of Artificial Sequence: Synthetic oligonucleotide"
  source 1..51: mol_type = other DNA
caagcagaagacggcatacgagatcagtgtagagatttggacctgcgagcg

SEQ ID NO: 448 - DNA, 51 bp, synthetic construct
  misc_feature 1..51: note = source = /note="Description of Artificial Sequence: Synthetic oligonucleotide"
  source 1..51: mol_type = other DNA
caagcagaagacggcatacgagatgattctcaagatttggacctgcgagcg

SEQ ID NO: 449 - DNA, 51 bp, synthetic construct
  misc_feature 1..51: note = source = /note="Description of Artificial Sequence: Synthetic oligonucleotide"
  source 1..51: mol_type = other DNA
caagcagaagacggcatacgagatccttcttaagatttggacctgcgagcg

SEQ ID NO: 450 - DNA, 51 bp, synthetic construct
  misc_feature 1..51: note = source = /note="Description of Artificial Sequence: Synthetic oligonucleotide"
  source 1..51: mol_type = other DNA
caagcagaagacggcatacgagattctaagacagatttggacctgcgagcg

SEQ ID NO: 451 - DNA, 51 bp, synthetic construct
  misc_feature 1..51: note = source = /note="Description of Artificial Sequence: Synthetic oligonucleotide"
  source 1..51: mol_type = other DNA
caagcagaagacggcatacgagatgcggcataagatttggacctgcgagcg

SEQ ID NO: 452 - DNA, 51 bp, synthetic construct
  misc_feature 1..51: note = source = /note="Description of Artificial Sequence: Synthetic oligonucleotide"
  source 1..51: mol_type = other DNA
caagcagaagacggcatacgagatattgacgaagatttggacctgcgagcg

SEQ ID NO: 453 - DNA, 51 bp, synthetic construct
  misc_feature 1..51: note = source = /note="Description of Artificial Sequence: Synthetic oligonucleotide"
  source 1..51: mol_type = other DNA
caagcagaagacggcatacgagatgctcctgaagatttggacctgcgagcg

SEQ ID NO: 454 - DNA, 51 bp, synthetic construct
  misc_feature 1..51: note = source = /note="Description of Artificial Sequence: Synthetic oligonucleotide"
  source 1..51: mol_type = other DNA
caagcagaagacggcatacgagatgcaatcctagatttggacctgcgagcg

SEQ ID NO: 455 - DNA, 51 bp, synthetic construct
  misc_feature 1..51: note = source = /note="Description of Artificial Sequence: Synthetic oligonucleotide"
  source 1..51: mol_type = other DNA
caagcagaagacggcatacgagatatgtcgttagatttggacctgcgagcg

SEQ ID NO: 456 - DNA, 51 bp, synthetic construct
  misc_feature 1..51: note = source = /note="Description of Artificial Sequence: Synthetic oligonucleotide"
  source 1..51: mol_type = other DNA
caagcagaagacggcatacgagatttctcggcagatttggacctgcgagcg

SEQ ID NO: 457 - DNA, 51 bp, synthetic construct
  misc_feature 1..51: note = source = /note="Description of Artificial Sequence: Synthetic oligonucleotide"
  source 1..51: mol_type = other DNA
caagcagaagacggcatacgagatcagggctaagatttggacctgcgagcg

SEQ ID NO: 458 - DNA, 51 bp, synthetic construct
  misc_feature 1..51: note = source = /note="Description of Artificial Sequence: Synthetic oligonucleotide"
  source 1..51: mol_type = other DNA
caagcagaagacggcatacgagatagccaagcagatttggacctgcgagcg

SEQ ID NO: 459 - DNA, 51 bp, synthetic construct
  misc_feature 1..51: note = source = /note="Description of Artificial Sequence: Synthetic oligonucleotide"
  source 1..51: mol_type = other DNA
caagcagaagacggcatacgagataagcctgaagatttggacctgcgagcg

SEQ ID NO: 460 - DNA, 51 bp, synthetic construct
  misc_feature 1..51: note = source = /note="Description of Artificial Sequence: Synthetic oligonucleotide"
  source 1..51: mol_type = other DNA
caagcagaagacggcatacgagatctacagagagatttggacctgcgagcg

SEQ ID NO: 461 - DNA, 51 bp, synthetic construct
  misc_feature 1..51: note = source = /note="Description of Artificial Sequence: Synthetic oligonucleotide"
  source 1..51: mol_type = other DNA
caagcagaagacggcatacgagatcgtagtcgagatttggacctgcgagcg

SEQ ID NO: 462 - DNA, 51 bp, synthetic construct
  misc_feature 1..51: note = source = /note="Description of Artificial Sequence: Synthetic oligonucleotide"
  source 1..51: mol_type = other DNA
caagcagaagacggcatacgagatttctgctcagatttggacctgcgagcg

SEQ ID NO: 463 - DNA, 51 bp, synthetic construct
  misc_feature 1..51: note = source = /note="Description of Artificial Sequence: Synthetic oligonucleotide"
  source 1..51: mol_type = other DNA
caagcagaagacggcatacgagatgtgcacacagatttggacctgcgagcg

SEQ ID NO: 464 - DNA, 51 bp, synthetic construct
  misc_feature 1..51: note = source = /note="Description of Artificial Sequence: Synthetic oligonucleotide"
  source 1..51: mol_type = other DNA
caagcagaagacggcatacgagataaagctcaagatttggacctgcgagcg

SEQ ID NO: 465 - DNA, 51 bp, synthetic construct
  misc_feature 1..51: note = source = /note="Description of Artificial Sequence: Synthetic oligonucleotide"
  source 1..51: mol_type = other DNA
caagcagaagacggcatacgagatgacctcagagatttggacctgcgagcg

SEQ ID NO: 466 - DNA, 51 bp, synthetic construct
  misc_feature 1..51: note = source = /note="Description of Artificial Sequence: Synthetic oligonucleotide"
  source 1..51: mol_type = other DNA
caagcagaagacggcatacgagatctttccaaagatttggacctgcgagcg

SEQ ID NO: 467 - DNA, 51 bp, synthetic construct
  misc_feature 1..51: note = source = /note="Description of Artificial Sequence: Synthetic oligonucleotide"
  source 1..51: mol_type = other DNA
caagcagaagacggcatacgagattcttggctagatttggacctgcgagcg

SEQ ID NO: 468 - DNA, 51 bp, synthetic construct
  misc_feature 1..51: note = source = /note="Description of Artificial Sequence: Synthetic oligonucleotide"
  source 1..51: mol_type = other DNA
caagcagaagacggcatacgagatcgcgtctaagatttggacctgcgagcg

SEQ ID NO: 469 - DNA, 51 bp, synthetic construct
  misc_feature 1..51: note = source = /note="Description of Artificial Sequence: Synthetic oligonucleotide"
  source 1..51: mol_type = other DNA
caagcagaagacggcatacgagattcgcgctaagatttggacctgcgagcg

SEQ ID NO: 470 - DNA, 51 bp, synthetic construct
  misc_feature 1..51: note = source = /note="Description of Artificial Sequence: Synthetic oligonucleotide"
  source 1..51: mol_type = other DNA
caagcagaagacggcatacgagatatccattcagatttggacctgcgagcg

SEQ ID NO: 471 - DNA, 51 bp, synthetic construct
  misc_feature 1..51: note = source = /note="Description of Artificial Sequence: Synthetic oligonucleotide"
  source 1..51: mol_type = other DNA
caagcagaagacggcatacgagatgcccagtaagatttggacctgcgagcg

SEQ ID NO: 472 - DNA, 51 bp, synthetic construct
  misc_feature 1..51: note = source = /note="Description of Artificial Sequence: Synthetic oligonucleotide"
  source 1..51: mol_type = other DNA
caagcagaagacggcatacgagattaccgacgagatttggacctgcgagcg

SEQ ID NO: 473 - DNA, 51 bp, synthetic construct
  misc_feature 1..51: note = source = /note="Description of Artificial Sequence: Synthetic oligonucleotide"
  source 1..51: mol_type = other DNA
caagcagaagacggcatacgagattccatacgagatttggacctgcgagcg

SEQ ID NO: 474 - DNA, 51 bp, synthetic construct
  misc_feature 1..51: note = source = /note="Description of Artificial Sequence: Synthetic oligonucleotide"
  source 1..51: mol_type = other DNA
caagcagaagacggcatacgagataacatgtcagatttggacctgcgagcg

SEQ ID NO: 475 - DNA, 51 bp, synthetic construct
  misc_feature 1..51: note = source = /note="Description of Artificial Sequence: Synthetic oligonucleotide"
  source 1..51: mol_type = other DNA
caagcagaagacggcatacgagatcgactataagatttggacctgcgagcg

SEQ ID NO: 476 - DNA, 51 bp, synthetic construct
  misc_feature 1..51: note = source = /note="Description of Artificial Sequence: Synthetic oligonucleotide"
  source 1..51: mol_type = other DNA
caagcagaagacggcatacgagatacccaaagagatttggacctgcgagcg

SEQ ID NO: 477 - DNA, 51 bp, synthetic construct
  misc_feature 1..51: note = source = /note="Description of Artificial Sequence: Synthetic oligonucleotide"
  source 1..51: mol_type = other DNA
caagcagaagacggcatacgagatatcgatcgagatttggacctgcgagcg

SEQ ID NO: 478 - DNA, 51 bp, synthetic construct
  misc_feature 1..51: note = source = /note="Description of Artificial Sequence: Synthetic oligonucleotide"
  source 1..51: mol_type = other DNA
caagcagaagacggcatacgagatgttggatgagatttggacctgcgagcg

SEQ ID NO: 479 - DNA, 51 bp, synthetic construct
  misc_feature 1..51: note = source = /note="Description of Artificial Sequence: Synthetic oligonucleotide"
  source 1..51: mol_type = other DNA
caagcagaagacggcatacgagatctatgtgaagatttggacctgcgagcg

SEQ ID NO: 480 - DNA, 51 bp, synthetic construct
  misc_feature 1..51: note = source = /note="Description of Artificial Sequence: Synthetic oligonucleotide"
  source 1..51: mol_type = other DNA
caagcagaagacggcatacgagattatttcgcagatttggacctgcgagcg

SEQ ID NO: 481 - DNA, 51 bp, synthetic construct
  misc_feature 1..51: note = source = /note="Description of Artificial Sequence: Synthetic oligonucleotide"
  source 1..51: mol_type = other DNA
caagcagaagacggcatacgagatccatgtatagatttggacctgcgagcg

SEQ ID NO: 482 - DNA, 51 bp, synthetic construct
  misc_feature 1..51: note = source = /note="Description of Artificial Sequence: Synthetic oligonucleotide"
  source 1..51: mol_type = other DNA
caagcagaagacggcatacgagatgccacgttagatttggacctgcgagcg

SEQ ID NO: 483 - DNA, 51 bp, synthetic construct
  misc_feature 1..51: note = source = /note="Description of Artificial Sequence: Synthetic oligonucleotide"
  source 1..51: mol_type = other DNA
caagcagaagacggcatacgagatgtcgtgtaagatttggacctgcgagcg

SEQ ID NO: 484 - DNA, 51 bp, synthetic construct
  misc_feature 1..51: note = source = /note="Description of Artificial Sequence: Synthetic oligonucleotide"
  source 1..51: mol_type = other DNA
caagcagaagacggcatacgagattaaagtcgagatttggacctgcgagcg

SEQ ID NO: 485 - DNA, 51 bp, synthetic construct
  misc_feature 1..51: note = source = /note="Description of Artificial Sequence: Synthetic oligonucleotide"
  source 1..51: mol_type = other DNA
caagcagaagacggcatacgagatcttcggacagatttggacctgcgagcg

SEQ ID NO: 486 - DNA, 51 bp, synthetic construct
  misc_feature 1..51: note = source = /note="Description of Artificial Sequence: Synthetic oligonucleotide"
  source 1..51: mol_type = other DNA
caagcagaagacggcatacgagatgcactctcagatttggacctgcgagcg

SEQ ID NO: 487 - DNA, 51 bp, synthetic construct
  misc_feature 1..51: note = source = /note="Description of Artificial Sequence: Synthetic oligonucleotide"
  source 1..51: mol_type = other DNA
caagcagaagacggcatacgagattcagatacagatttggacctgcgagcg

SEQ ID NO: 488 - DNA, 51 bp, synthetic construct
  misc_feature 1..51: note = source = /note="Description of Artificial Sequence: Synthetic oligonucleotide"
  source 1..51: mol_type = other DNA
caagcagaagacggcatacgagatcagtccctagatttggacctgcgagcg

SEQ ID NO: 489 - DNA, 51 bp, synthetic construct
  misc_feature 1..51: note = source = /note="Description of Artificial Sequence: Synthetic oligonucleotide"
  source 1..51: mol_type = other DNA
caagcagaagacggcatacgagatgccctaacagatttggacctgcgagcg

SEQ ID NO: 490 - DNA, 51 bp, synthetic construct
  misc_feature 1..51: note = source = /note="Description of Artificial Sequence: Synthetic oligonucleotide"
  source 1..51: mol_type = other DNA
caagcagaagacggcatacgagatctgcatcaagatttggacctgcgagcg

SEQ ID NO: 491 - DNA, 51 bp, synthetic construct
  misc_feature 1..51: note = source = /note="Description of Artificial Sequence: Synthetic oligonucleotide"
  source 1..51: mol_type = other DNA
caagcagaagacggcatacgagatcggtatcgagatttggacctgcgagcg

SEQ ID NO: 492 - DNA, 51 bp, synthetic construct
  misc_feature 1..51: note = source = /note="Description of Artificial Sequence: Synthetic oligonucleotide"
  source 1..51: mol_type = other DNA
caagcagaagacggcatacgagataagtatggagatttggacctgcgagcg

SEQ ID NO: 493 - DNA, 51 bp, synthetic construct
  misc_feature 1..51: note = source = /note="Description of Artificial Sequence: Synthetic oligonucleotide"
  source 1..51: mol_type = other DNA
caagcagaagacggcatacgagatattcgcgcagatttggacctgcgagcg

SEQ ID NO: 494 - DNA, 51 bp, synthetic construct
  misc_feature 1..51: note = source = /note="Description of Artificial Sequence: Synthetic oligonucleotide"
  source 1..51: mol_type = other DNA
caagcagaagacggcatacgagatatcaaggtagatttggacctgcgagcg

SEQ ID NO: 495 - DNA, 51 bp, synthetic construct
  misc_feature 1..51: note = source = /note="Description of Artificial Sequence: Synthetic oligonucleotide"
  source 1..51: mol_type = other DNA
caagcagaagacggcatacgagatttgtgcatagatttggacctgcgagcg

SEQ ID NO: 496 - DNA, 51 bp, synthetic construct
  misc_feature 1..51: note = source = /note="Description of Artificial Sequence: Synthetic oligonucleotide"
  source 1..51: mol_type = other DNA
caagcagaagacggcatacgagatctgtgctgagatttggacctgcgagcg

SEQ ID NO: 497 - DNA, 51 bp, synthetic construct
  misc_feature 1..51: note = source = /note="Description of Artificial Sequence: Synthetic oligonucleotide"
  source 1..51: mol_type = other DNA
caagcagaagacggcatacgagatgtccgtagagatttggacctgcgagcg

SEQ ID NO: 498 - DNA, 51 bp, synthetic construct
  misc_feature 1..51: note = source = /note="Description of Artificial Sequence: Synthetic oligonucleotide"
  source 1..51: mol_type = other DNA
caagcagaagacggcatacgagatgttcaagaagatttggacctgcgagcg

SEQ ID NO: 499 - DNA, 51 bp, synthetic construct
  misc_feature 1..51: note = source = /note="Description of Artificial Sequence: Synthetic oligonucleotide"
  source 1..51: mol_type = other DNA
caagcagaagacggcatacgagatcaccgttcagatttggacctgcgagcg

SEQ ID NO: 500 - DNA, 51 bp, synthetic construct
  misc_feature 1..51: note = source = /note="Description of Artificial Sequence: Synthetic oligonucleotide"
  source 1..51: mol_type = other DNA
caagcagaagacggcatacgagatcgagttgaagatttggacctgcgagcg

SEQ ID NO: 501 - DNA, 51 bp, synthetic construct
  misc_feature 1..51: note = source = /note="Description of Artificial Sequence: Synthetic oligonucleotide"
  source 1..51: mol_type = other DNA
caagcagaagacggcatacgagatgagcacgaagatttggacctgcgagcg

SEQ ID NO: 502 - DNA, 51 bp, synthetic construct
  misc_feature 1..51: note = source = /note="Description of Artificial Sequence: Synthetic oligonucleotide"
  source 1..51: mol_type = other DNA
caagcagaagacggcatacgagatagttcgtgagatttggacctgcgagcg

SEQ ID NO: 503 - DNA, 51 bp, synthetic construct
  misc_feature 1..51: note = source = /note="Description of Artificial Sequence: Synthetic oligonucleotide"
  source 1..51: mol_type = other DNA
caagcagaagacggcatacgagatcatcaactagatttggacctgcgagcg

SEQ ID NO: 504 - DNA, 51 bp, synthetic construct
  misc_feature 1..51: note = source = /note="Description of Artificial Sequence: Synthetic oligonucleotide"
  source 1..51: mol_type = other DNA
caagcagaagacggcatacgagatcgagatctagatttggacctgcgagcg

SEQ ID NO: 505 - DNA, 51 bp, synthetic construct
  misc_feature 1..51: note = source = /note="Description of Artificial Sequence: Synthetic oligonucleotide"
  source 1..51: mol_type = other DNA
caagcagaagacggcatacgagattggccagaagatttggacctgcgagcg

SEQ ID NO: 506 - DNA, 51 bp, synthetic construct
  misc_feature 1..51: note = source = /note="Description of Artificial Sequence: Synthetic oligonucleotide"
  source 1..51: mol_type = other DNA
caagcagaagacggcatacgagatttcaccatagatttggacctgcgagcg

SEQ ID NO: 507 - DNA, 51 bp, synthetic construct
  misc_feature 1..51: note = source = /note="Description of Artificial Sequence: Synthetic oligonucleotide"
  source 1..51: mol_type = other DNA
caagcagaagacggcatacgagatgaatgcatagatttggacctgcgagcg

SEQ ID NO: 508 - DNA, 51 bp, synthetic construct
  misc_feature 1..51: note = source = /note="Description of Artificial Sequence: Synthetic oligonucleotide"
  source 1..51: mol_type = other DNA
caagcagaagacggcatacgagattggaccctagatttggacctgcgagcg

SEQ ID NO: 509 - DNA, 51 bp, synthetic construct
  misc_feature 1..51: note = source = /note="Description of Artificial Sequence: Synthetic oligonucleotide"
  source 1..51: mol_type = other DNA
caagcagaagacggcatacgagatgatagcacagatttggacctgcgagcg

SEQ ID NO: 510 - DNA, 51 bp, synthetic construct
  misc_feature 1..51: note = source = /note="Description of Artificial Sequence: Synthetic oligonucleotide"
  source 1..51: mol_type = other DNA
caagcagaagacggcatacgagatacgacgacagatttggacctgcgagcg

SEQ ID NO: 511 - DNA, 51 bp, synthetic construct
  misc_feature 1..51: note = source = /note="Description of Artificial Sequence: Synthetic oligonucleotide"
  source 1..51: mol_type = other DNA
caagcagaagacggcatacgagatctcagtatagatttggacctgcgagcg

SEQ ID NO: 512 - DNA, 51 bp, synthetic construct
  misc_feature 1..51: note = source = /note="Description of Artificial Sequence: Synthetic oligonucleotide"
  source 1..51: mol_type = other DNA
caagcagaagacggcatacgagatcttagctaagatttggacctgcgagcg

SEQ ID NO: 513 - DNA, 51 bp, synthetic construct
  misc_feature 1..51: note = source = /note="Description of Artificial Sequence: Synthetic oligonucleotide"
  source 1..51: mol_type = other DNA
caagcagaagacggcatacgagatctgtttacagatttggacctgcgagcg

SEQ ID NO: 514 - DNA, 51 bp, synthetic construct
  misc_feature 1..51: note = source = /note="Description of Artificial Sequence: Synthetic oligonucleotide"
  source 1..51: mol_type = other DNA
caagcagaagacggcatacgagattgtcccacagatttggacctgcgagcg

SEQ ID NO: 515 - DNA, 51 bp, synthetic construct
  misc_feature 1..51: note = source = /note="Description of Artificial Sequence: Synthetic oligonucleotide"
  source 1..51: mol_type = other DNA
caagcagaagacggcatacgagattcctgaggagatttggacctgcgagcg

SEQ ID NO: 516 - DNA, 51 bp, synthetic construct
  misc_feature 1..51: note = source = /note="Description of Artificial Sequence: Synthetic oligonucleotide"
  source 1..51: mol_type = other DNA
caagcagaagacggcatacgagattagttccaagatttggacctgcgagcg

SEQ ID NO: 517 - DNA, 51 bp, synthetic construct
  misc_feature 1..51: note = source = /note="Description of Artificial Sequence: Synthetic oligonucleotide"
  source 1..51: mol_type = other DNA
caagcagaagacggcatacgagatcatgactcagatttggacctgcgagcg

SEQ ID NO: 518 - DNA, 51 bp, synthetic construct
  misc_feature 1..51: note = source = /note="Description of Artificial Sequence: Synthetic oligonucleotide"
  source 1..51: mol_type = other DNA
caagcagaagacggcatacgagatgtaagcgcagatttggacctgcgagcg

SEQ ID NO: 519 - DNA, 51 bp, synthetic construct
  misc_feature 1..51: note = source = /note="Description of Artificial Sequence: Synthetic oligonucleotide"
  source 1..51: mol_type = other DNA
caagcagaagacggcatacgagataacccagtagatttggacctgcgagcg

SEQ ID NO: 520 - DNA, 51 bp, synthetic construct
  misc_feature 1..51: note = source = /note="Description of Artificial Sequence: Synthetic oligonucleotide"
  source 1..51: mol_type = other DNA
caagcagaagacggcatacgagattttgagggagatttggacctgcgagcg

SEQ ID NO: 521 - DNA, 51 bp, synthetic construct
  misc_feature 1..51: note = source = /note="Description of Artificial Sequence: Synthetic oligonucleotide"
  source 1..51: mol_type = other DNA
caagcagaagacggcatacgagatagccgacaagatttggacctgcgagcg

SEQ ID NO: 522 - DNA, 51 bp, synthetic construct
  misc_feature 1..51: note = source = /note="Description of Artificial Sequence: Synthetic oligonucleotide"
  source 1..51: mol_type = other DNA
caagcagaagacggcatacgagataaacccgcagatttggacctgcgagcg

SEQ ID NO: 523 - DNA, 51 bp, synthetic construct
  misc_feature 1..51: note = source = /note="Description of Artificial Sequence: Synthetic oligonucleotide"
  source 1..51: mol_type = other DNA
caagcagaagacggcatacgagatgtagggctagatttggacctgcgagcg

SEQ ID NO: 524 - DNA, 51 bp, synthetic construct
  misc_feature 1..51: note = source = /note="Description of Artificial Sequence: Synthetic oligonucleotide"
  source 1..51: mol_type = other DNA
caagcagaagacggcatacgagatagacgattagatttggacctgcgagcg

SEQ ID NO: 525 - DNA, 51 bp, synthetic construct
  misc_feature 1..51: note = source = /note="Description of Artificial Sequence: Synthetic oligonucleotide"
  source 1..51: mol_type = other DNA
caagcagaagacggcatacgagataggatgatagatttggacctgcgagcg

SEQ ID NO: 526 - DNA, 51 bp, synthetic construct
  misc_feature 1..51: note = source = /note="Description of Artificial Sequence: Synthetic oligonucleotide"
  source 1..51: mol_type = other DNA
caagcagaagacggcatacgagatataatggcagatttggacctgcgagcg

SEQ ID NO: 527 - DNA, 51 bp, synthetic construct
  misc_feature 1..51: note = source = /note="Description of Artificial Sequence: Synthetic oligonucleotide"
  source 1..51: mol_type = other DNA
caagcagaagacggcatacgagatcttggcgtagatttggacctgcgagcg

SEQ ID NO: 528 - DNA, 51 bp, synthetic construct
  misc_feature 1..51: note = source = /note="Description of Artificial Sequence: Synthetic oligonucleotide"
  source 1..51: mol_type = other DNA
caagcagaagacggcatacgagatagctgtgcagatttggacctgcgagcg

SEQ ID NO: 529 - DNA, 51 bp, synthetic construct
  misc_feature 1..51: note = source = /note="Description of Artificial Sequence: Synthetic oligonucleotide"
  source 1..51: mol_type = other DNA
caagcagaagacggcatacgagatgagtccaaagatttggacctgcgagcg

SEQ ID NO: 530 - DNA, 51 bp, synthetic construct
  misc_feature 1..51: note = source = /note="Description of Artificial Sequence: Synthetic oligonucleotide"
  source 1..51: mol_type = other DNA
caagcagaagacggcatacgagatgaataccaagatttggacctgcgagcg

SEQ ID NO: 531 - DNA, 51 bp, synthetic construct
  misc_feature 1..51: note = source = /note="Description of Artificial Sequence: Synthetic oligonucleotide"
  source 1..51: mol_type = other DNA
caagcagaagacggcatacgagataggagcttagatttggacctgcgagcg

SEQ ID NO: 532 - DNA, 51 bp, synthetic construct
  misc_feature 1..51: note = source = /note="Description of Artificial Sequence: Synthetic oligonucleotide"
  source 1..51: mol_type = other DNA
caagcagaagacggcatacgagatgtgacttaagatttggacctgcgagcg

SEQ ID NO: 533 - DNA, 51 bp, synthetic construct
  misc_feature 1..51: note = source = /note="Description of Artificial Sequence: Synthetic oligonucleotide"
  source 1..51: mol_type = other DNA
caagcagaagacggcatacgagattttggaacagatttggacctgcgagcg

SEQ ID NO: 534 - DNA, 57 bp, synthetic construct
  misc_feature 1..57: note = source = /note="Description of Artificial Sequence: Synthetic oligonucleotide"
  source 1..57: mol_type = other DNA
aatgatacggcgaccaccgagatctacacctctctatgagcggctgtctccacaagt

SEQ ID NO: 535 - DNA, 57 bp, synthetic construct
  misc_feature 1..57: note = source = /note="Description of Artificial Sequence: Synthetic oligonucleotide"
  source 1..57: mol_type = other DNA
aatgatacggcgaccaccgagatctacactatcctctgagcggctgtctccacaagt

SEQ ID NO: 536 - DNA, 57 bp, synthetic construct
  misc_feature 1..57: note = source = /note="Description of Artificial Sequence: Synthetic oligonucleotide"
  source 1..57: mol_type = other DNA
aatgatacggcgaccaccgagatctacacgtaaggaggagcggctgtctccacaagt

SEQ ID NO: 537 - DNA, 57 bp, synthetic construct
  misc_feature 1..57: note = source = /note="Description of Artificial Sequence: Synthetic oligonucleotide"
  source 1..57: mol_type = other DNA
aatgatacggcgaccaccgagatctacacactgcatagagcggctgtctccacaagt

SEQ ID NO: 538 - DNA, 48 bp, synthetic construct
  misc_feature 1..48: note = source = /note="Description of Artificial Sequence: Synthetic oligonucleotide"
  source 1..48: mol_type = other DNA
aatgatacggcgaccaccgaaaggagtagagcggctgtctccacaagt

SEQ ID NO: 539 - DNA, 48 bp, synthetic construct
  misc_feature 1..48: note = source = /note="Description of Artificial Sequence: Synthetic oligonucleotide"
  source 1..48: mol_type = other DNA
aatgatacggcgaccaccgactaagcctgagcggctgtctccacaagt

SEQ ID NO: 540 - DNA, 48 bp, synthetic construct
  misc_feature 1..48: note = source = /note="Description of Artificial Sequence: Synthetic oligonucleotide"
  source 1..48: mol_type = other DNA
aatgatacggcgaccaccgacgtctaatgagcggctgtctccacaagt

SEQ ID NO: 541 - DNA, 48 bp, synthetic construct
  misc_feature 1..48: note = source = /note="Description of Artificial Sequence: Synthetic oligonucleotide"
  source 1..48: mol_type = other DNA
aatgatacggcgaccaccgatctctccggagcggctgtctccacaagt

SEQ ID NO: 542 - DNA, 57 bp, synthetic construct; identical to SEQ ID NO: 114
  misc_feature 1..57: note = source = /note="Description of Artificial Sequence: Synthetic oligonucleotide"
  source 1..57: mol_type = other DNA

SEQ ID NO: 543 - DNA, 57 bp, synthetic construct
  misc_feature 1..57: note = source = /note="Description of Artificial Sequence: Synthetic oligonucleotide"
  source 1..57: mol_type = other DNA
aatgatacggcgaccaccgagatctacactgtcatgagagcggctgtctccacaagt

SEQ ID NO: 544 - DNA, 57 bp, synthetic construct
  misc_feature 1..57: note = source = /note="Description of Artificial Sequence: Synthetic oligonucleotide"
  source 1..57: mol_type = other DNA
aatgatacggcgaccaccgagatctacactgtaacaggagcggctgtctccacaagt

SEQ ID NO: 545 - DNA, 57 bp, synthetic construct
  misc_feature 1..57: note = source = /note="Description of Artificial Sequence: Synthetic oligonucleotide"
  source 1..57: mol_type = other DNA
aatgatacggcgaccaccgagatctacacgcgcaactgagcggctgtctccacaagt

SEQ ID NO: 546 - DNA, 48 bp, synthetic construct
  misc_feature 1..48: note = source = /note="Description of Artificial Sequence: Synthetic oligonucleotide"
  source 1..48: mol_type = other DNA
aatgatacggcgaccaccgatcgatggcgagcggctgtctccacaagt

SEQ ID NO: 547 - DNA, 48 bp, synthetic construct
  misc_feature 1..48: note = source = /note="Description of Artificial Sequence: Synthetic oligonucleotide"
  source 1..48: mol_type = other DNA
aatgatacggcgaccaccgacatggtttgagcggctgtctccacaagt

SEQ ID NO: 548 - DNA, 48 bp, synthetic construct
  misc_feature 1..48: note = source = /note="Description of Artificial Sequence: Synthetic oligonucleotide"
  source 1..48: mol_type = other DNA
aatgatacggcgaccaccgaacgaaagcgagcggctgtctccacaagt

SEQ ID NO: 549 - DNA, 48 bp, synthetic construct
  misc_feature 1..48: note = source = /note="Description of Artificial Sequence: Synthetic oligonucleotide"
  source 1..48: mol_type = other DNA
aatgatacggcgaccaccgagctctgatgagcggctgtctccacaagt

SEQ ID NO: 550 - DNA, 57 bp, synthetic construct
  misc_feature 1..57: note = source = /note="Description of Artificial Sequence: Synthetic oligonucleotide"
  source 1..57: mol_type = other DNA
aatgatacggcgaccaccgagatctacacatgccctcgagcggctgtctccacaagt

SEQ ID NO: 551 - DNA, 57 bp, synthetic construct
  misc_feature 1..57: note = source = /note="Description of Artificial Sequence: Synthetic oligonucleotide"
  source 1..57: mol_type = other DNA
aatgatacggcgaccaccgagatctacacctcagatggagcggctgtctccacaagt

SEQ ID NO: 552 - DNA, 57 bp, synthetic construct
  misc_feature 1..57: note = source = /note="Description of Artificial Sequence: Synthetic oligonucleotide"
  source 1..57: mol_type = other DNA
aatgatacggcgaccaccgagatctacacgtaatctggagcggctgtctccacaagt

SEQ ID NO: 553 - DNA, 57 bp, synthetic construct
  misc_feature 1..57: note = source = /note="Description of Artificial Sequence: Synthetic oligonucleotide"
  source 1..57: mol_type = other DNA
aatgatacggcgaccaccgagatctacacgcaagattgagcggctgtctccacaagt

SEQ ID NO: 554 - DNA, 48 bp, synthetic construct
  misc_feature 1..48: note = source = /note="Description of Artificial Sequence: Synthetic oligonucleotide"
  source 1..48: mol_type = other DNA
aatgatacggcgaccaccgaatacgccagagcggctgtctccacaagt

SEQ ID NO: 555 - DNA, 48 bp, synthetic construct
  misc_feature 1..48: note = source = /note="Description of Artificial Sequence: Synthetic oligonucleotide"
  source 1..48: mol_type = other DNA
aatgatacggcgaccaccgaaccagtcggagcggctgtctccacaagt

SEQ ID NO: 556 - DNA, 48 bp, synthetic construct
  misc_feature 1..48: note = source = /note="Description of Artificial Sequence: Synthetic oligonucleotide"
  source 1..48: mol_type = other DNA
aatgatacggcgaccaccgaaacacggagagcggctgtctccacaagt

SEQ ID NO: 557 - DNA, 48 bp, synthetic construct
  misc_feature 1..48: note = source = /note="Description of Artificial Sequence: Synthetic oligonucleotide"
  source 1..48: mol_type = other DNA
aatgatacggcgaccaccgactgcctaggagcggctgtctccacaagt

SEQ ID NO: 558 - DNA, 43 bp, synthetic construct
  misc_feature 1..43: note = source = /note="Description of Artificial Sequence: Synthetic oligonucleotide"
  source 1..43: mol_type = other DNA
gggtcacgcgtaggagttctatcgaccccaaaatcagcgaaat

SEQ ID NO: 559 - DNA, 47 bp, synthetic construct
  misc_feature 1..47: note = source = /note="Description of Artificial Sequence: Synthetic oligonucleotide"
  source 1..47: mol_type = other DNA
gttccgcagccacacaagatctgtctggttactgccagttgaatctg

SEQ ID NO: 560 - DNA, 43 bp, synthetic construct
  misc_feature 1..43: note = source = /note="Description of Artificial Sequence: Synthetic oligonucleotide"
  source 1..43: mol_type = other DNA
cgcgtcgagtagggtgttctatcgaccccaaaatcagcgaaat

SEQ ID NO: 561 - DNA, 47 bp, synthetic construct
  misc_feature 1..47: note = source = /note="Description of Artificial Sequence: Synthetic oligonucleotide"
  source 1..47: mol_type = other DNA
gccgtgtgaagctggaagatctgtctggttactgccagttgaatctg

SEQ ID NO: 562 - DNA, 43 bp, synthetic construct
  misc_feature 1..43: note = source = /note="Description of Artificial Sequence: Synthetic oligonucleotide"
  source 1..43: mol_type = other DNA
cgatcgcccttggtggttctatcgaccccaaaatcagcgaaat

SEQ ID NO: 563 - DNA, 47 bp, synthetic construct
  misc_feature 1..47: note = source = /note="Description of Artificial Sequence: Synthetic oligonucleotide"
  source 1..47: mol_type = other DNA
ggtttagccggcgtgaagatctgtctggttactgccagttgaatctg

SEQ ID NO: 564 - DNA, 43 bp, synthetic construct
  misc_feature 1..43: note = source = /note="Description of Artificial Sequence: Synthetic oligonucleotide"
  source 1..43: mol_type = other DNA
ggtcgagccggaactgttctatcgaccccaaaatcagcgaaat

SEQ ID NO: 565 - DNA, 47 bp, synthetic construct
  misc_feature 1..47: note = source = /note="Description of Artificial Sequence: Synthetic oligonucleotide"
  source 1..47: mol_type = other DNA
ggatgcgcacccagaaagatctgtctggttactgccagttgaatctg

SEQ ID NO: 566 - DNA, 43 bp, synthetic construct
  misc_feature 1..43: note = source = /note="Description of Artificial Sequence: Synthetic oligonucleotide"
  source 1..43: mol_type = other DNA
tcccggcgttgtcctgttctatcgaccccaaaatcagcgaaat

SEQ ID NO: 567 - DNA, 47 bp, synthetic construct
  misc_feature 1..47: note = source = /note="Description of Artificial Sequence: Synthetic oligonucleotide"
  source 1..47: mol_type = other DNA
gctccgtcactgcccaagatctgtctggttactgccagttgaatctg

SEQ ID NO: 568 - DNA, 43 bp, synthetic construct
  misc_feature 1..43: note = source = /note="Description of Artificial Sequence: Synthetic oligonucleotide"
  source 1..43: mol_type = other DNA
cgcagggtccagagtgttctatcgaccccaaaatcagcgaaat

SEQ ID NO: 569 - DNA, 47 bp, synthetic construct
  misc_feature 1..47: note = source = /note="Description of Artificial Sequence: Synthetic oligonucleotide"
  source 1..47: mol_type = other DNA
gttcgcgcgaaggaaaagatctgtctggttactgccagttgaatctg

SEQ ID NO: 570 - DNA, 48 bp, synthetic construct
  misc_feature 1..48: note = source = /note="Description of Artificial Sequence: Synthetic oligonucleotide"
  source 1..48: mol_type = other DNA
atatagatgccgtcctagcggttctatcgaccccaaaatcagcgaaat

SEQ ID NO: 571 - DNA, 52 bp, synthetic construct
  misc_feature 1..52: note = source = /note="Description of Artificial Sequence: Synthetic oligonucleotide"
  source 1..52: mol_type = other DNA
aagtatctttcctgtgcccaaagatctgtctggttactgccagttgaatctg

SEQ ID NO: 572 - DNA, 48 bp, synthetic construct
  misc_feature 1..48: note = source = /note="Description of Artificial Sequence: Synthetic oligonucleotide"
  source 1..48: mol_type = other DNA
ccctttaatcagatgcgtcggttctatcgaccccaaaatcagcgaaat

SEQ ID NO: 573 - DNA, 52 bp, synthetic construct
  misc_feature 1..52: note = source = /note="Description of Artificial Sequence: Synthetic oligonucleotide"
  source 1..52: mol_type = other DNA
tggtagtaataagggcgaccaagatctgtctggttactgccagttgaatctg

SEQ ID NO: 574 - DNA, 48 bp, synthetic construct
  misc_feature 1..48: note = source = /note="Description of Artificial Sequence: Synthetic oligonucleotide"
  source 1..48: mol_type = other DNA
ttggtcatgtgcttttcgttgttctatcgaccccaaaatcagcgaaat

SEQ ID NO: 575 - DNA, 52 bp, synthetic construct
  misc_feature 1..52: note = source = /note="Description of Artificial Sequence: Synthetic oligonucleotide"
  source 1..52: mol_type = other DNA
aggggtatcggatactcagaaagatctgtctggttactgccagttgaatctg

SEQ ID NO: 576 - DNA, 48 bp, synthetic construct
  misc_feature 1..48: note = source = /note="Description of Artificial Sequence: Synthetic oligonucleotide"
  source 1..48: mol_type = other DNA
gggtgggtaaatggtaatgcgttctatcgaccccaaaatcagcgaaat

SEQ ID NO: 577 - DNA, 52 bp, synthetic construct
  misc_feature 1..52: note = source = /note="Description of Artificial Sequence: Synthetic oligonucleotide"
  source 1..52: mol_type = other DNA
atcgattccccggatatagcaagatctgtctggttactgccagttgaatctg

SEQ ID NO: 578 - DNA, 48 bp, synthetic construct
  misc_feature 1..48: note = source = /note="Description of Artificial Sequence: Synthetic oligonucleotide"
  source 1..48: mol_type = other DNA
tccgacggggagtatatactgttctatcgaccccaaaatcagcgaaat

SEQ ID NO: 579 - DNA, 52 bp, synthetic construct
  misc_feature 1..52: note = source = /note="Description of Artificial Sequence: Synthetic oligonucleotide"
  source 1..52: mol_type = other DNA
tactaactgcttcaggccaaaagatctgtctggttactgccagttgaatctg

SEQ ID NO: 580 - DNA, 48 bp, synthetic construct
  misc_feature 1..48: note = source = /note="Description of Artificial Sequence: Synthetic oligonucleotide"
  source 1..48: mol_type = other DNA
catgtttaggaacgctaccggttctatcgaccccaaaatcagcgaaat

SEQ ID NO: 581 - DNA, 52 bp, synthetic construct
  misc_feature 1..52: note = source = /note="Description of Artificial Sequence: Synthetic oligonucleotide"
  source 1..52: mol_type = other DNA
aataatctccgttccctcccaagatctgtctggttactgccagttgaatctg

SEQ ID NO: 582 - DNA, 43 bp, synthetic construct
  misc_feature 1..43: note = source = /note="Description of Artificial Sequence: Synthetic oligonucleotide"
  source 1..43: mol_type = other DNA
gggtcacgcgtaggagttctatcgctggtgctgcagcttatta

SEQ ID NO: 583 - DNA, 43 bp, synthetic construct
  misc_feature 1..43: note = source = /note="Description of Artificial Sequence: Synthetic oligonucleotide"
  source 1..43: mol_type = other DNA
gttccgcagccacacaagatctgagggtcaagtgcacagtcta

SEQ ID NO: 584 - DNA, 43 bp, synthetic construct
  misc_feature 1..43: note = source = /note="Description of Artificial Sequence: Synthetic oligonucleotide"
  source 1..43: mol_type = other DNA
cgcgtcgagtagggtgttctatcgctggtgctgcagcttatta

SEQ ID NO: 585 - DNA, 43 bp, synthetic construct
  misc_feature 1..43: note = source = /note="Description of Artificial Sequence: Synthetic oligonucleotide"
  source 1..43: mol_type = other DNA
gccgtgtgaagctggaagatctgagggtcaagtgcacagtcta

SEQ ID NO: 586 - DNA, 43 bp, synthetic construct
  misc_feature 1..43: note = source = /note="Description of Artificial Sequence: Synthetic oligonucleotide"
  source 1..43: mol_type = other DNA
cgatcgcccttggtggttctatcgctggtgctgcagcttatta

SEQ ID NO: 587 - DNA, 43 bp, synthetic construct
  misc_feature 1..43: note = source = /note="Description of Artificial Sequence: Synthetic oligonucleotide"
  source 1..43: mol_type = other DNA
ggtttagccggcgtgaagatctgagggtcaagtgcacagtcta

SEQ ID NO: 588 - DNA, 43 bp, synthetic construct
  misc_feature 1..43: note = source = /note="Description of Artificial Sequence: Synthetic oligonucleotide"
  source 1..43: mol_type = other DNA
ggtcgagccggaactgttctatcgctggtgctgcagcttatta

SEQ ID NO: 589 - DNA, 43 bp, synthetic construct
  misc_feature 1..43: note = source = /note="Description of Artificial Sequence: Synthetic oligonucleotide"
  source 1..43: mol_type = other DNA
ggatgcgcacccagaaagatctgagggtcaagtgcacagtcta

SEQ ID NO: 590 - DNA, 43 bp, synthetic construct
  misc_feature 1..43: note = source = /note="Description of Artificial Sequence: Synthetic oligonucleotide"
  source 1..43: mol_type = other DNA
tcccggcgttgtcctgttctatcgctggtgctgcagcttatta

SEQ ID NO: 591 - DNA, 43 bp, synthetic construct
  misc_feature 1..43: note = source = /note="Description of Artificial Sequence: Synthetic oligonucleotide"
  source 1..43: mol_type = other DNA
gctccgtcactgcccaagatctgagggtcaagtgcacagtcta

SEQ ID NO: 592 - DNA, 43 bp, synthetic construct
  misc_feature 1..43: note = source = /note="Description of Artificial Sequence: Synthetic oligonucleotide"
  source 1..43: mol_type = other DNA
cgcagggtccagagtgttctatcgctggtgctgcagcttatta

SEQ ID NO: 593 - DNA, 43 bp, synthetic construct
  misc_feature 1..43: note = source = /note="Description of Artificial Sequence: Synthetic oligonucleotide"
  source 1..43: mol_type = other DNA
gttcgcgcgaaggaaaagatctgagggtcaagtgcacagtcta

SEQ ID NO: 594 - DNA, 48 bp, synthetic construct
  misc_feature 1..48: note = source = /note="Description of Artificial Sequence: Synthetic oligonucleotide"
  source 1..48: mol_type = other DNA
atatagatgccgtcctagcggttctatcgctggtgctgcagcttatta

SEQ ID NO: 595 - DNA, 48 bp, synthetic construct
  misc_feature 1..48: note = source = /note="Description of Artificial Sequence: Synthetic oligonucleotide"
  source 1..48: mol_type = other DNA
aagtatctttcctgtgcccaaagatctgagggtcaagtgcacagtcta

SEQ ID NO: 596 - DNA, 48 bp, synthetic construct
  misc_feature 1..48: note = source = /note="Description of Artificial Sequence: Synthetic oligonucleotide"
  source 1..48: mol_type = other DNA
ccctttaatcagatgcgtcggttctatcgctggtgctgcagcttatta

SEQ ID NO: 597 - DNA, 48 bp, synthetic construct
  misc_feature 1..48: note = source = /note="Description of Artificial Sequence: Synthetic oligonucleotide"
  source 1..48: mol_type = other DNA
tggtagtaataagggcgaccaagatctgagggtcaagtgcacagtcta

SEQ ID NO: 598 - DNA, 48 bp, synthetic construct
  misc_feature 1..48: note = source = /note="Description of Artificial Sequence: Synthetic oligonucleotide"
  source 1..48: mol_type = other DNA
ttggtcatgtgcttttcgttgttctatcgctggtgctgcagcttatta

SEQ ID NO: 599 - DNA, 48 bp, synthetic construct
  misc_feature 1..48: note = source = /note="Description of Artificial Sequence: Synthetic oligonucleotide"
  source 1..48: mol_type = other DNA
aggggtatcggatactcagaaagatctgagggtcaagtgcacagtcta

SEQ ID NO: 600 - DNA, 48 bp, synthetic construct
  misc_feature 1..48: note = source = /note="Description of Artificial Sequence: Synthetic oligonucleotide"
  source 1..48: mol_type = other DNA
gggtgggtaaatggtaatgcgttctatcgctggtgctgcagcttatta

SEQ ID NO: 601 - DNA, 48 bp, synthetic construct
  misc_feature 1..48: note = source = /note="Description of Artificial Sequence: Synthetic oligonucleotide"
  source 1..48: mol_type = other DNA
atcgattccccggatatagcaagatctgagggtcaagtgcacagtcta

SEQ ID NO: 602 - DNA, 48 bp, synthetic construct
  misc_feature 1..48: note = source = /note="Description of Artificial Sequence: Synthetic oligonucleotide"
  source 1..48: mol_type = other DNA
tccgacggggagtatatactgttctatcgctggtgctgcagcttatta

SEQ ID NO: 603 - DNA, 48 bp, synthetic construct
  misc_feature 1..48: note = source = /note="Description of Artificial Sequence: Synthetic oligonucleotide"
  source 1..48: mol_type = other DNA
tactaactgcttcaggccaaaagatctgagggtcaagtgcacagtcta

SEQ ID NO: 604 - DNA, 48 bp, synthetic construct
  misc_feature 1..48: note = source = /note="Description of Artificial Sequence: Synthetic oligonucleotide"
  source 1..48: mol_type = other DNA
catgtttaggaacgctaccggttctatcgctggtgctgcagcttatta

SEQ ID NO: 605 - DNA, 48 bp, synthetic construct
  misc_feature 1..48: note = source = /note="Description of Artificial Sequence: Synthetic oligonucleotide"
  source 1..48: mol_type = other DNA
aataatctccgttccctcccaagatctgagggtcaagtgcacagtcta

SEQ ID NO: 606 - DNA, 108 bp, synthetic construct
  misc_feature 1..108: note = source = /note="Description of Artificial Sequence: Synthetic polynucleotide"
  source 1..108: mol_type = other DNA
gctggtgctgcagcttattatgtgggtgtgtatctcacgaagcgaccctttggaaaatataatgaaaatggaaccattacagatgctgtagactgtgcacttgaccct

SEQ ID NO: 607 - DNA, 108 bp, synthetic construct
  misc_feature 1..108: note = source = /note="Description of Artificial Sequence: Synthetic polynucleotide"
  source 1..108: mol_type = other DNA
gctggtgctgcagcttattatgtgggtcctcgctaggacgtcgctatgacgccaaaatataatgaaaatggaaccattacagatgctgtagactgtgcacttgaccct

SEQ ID NO: 608 - DNA, 108 bp, synthetic construct
  misc_feature 1..108: note = source = /note="Description of Artificial Sequence: Synthetic polynucleotide"
  source 1..108: mol_type = other DNA
gctggtgctgcagcttattatgtgggtagcacgacttgatctaactgacactaaaaatataatgaaaatggaaccattacagatgctgtagactgtgcacttgaccct

SEQ ID NO: 609 - DNA, 108 bp, synthetic construct
  misc_feature 1..108: note = source = /note="Description of Artificial Sequence: Synthetic polynucleotide"
  source 1..108: mol_type = other DNA
gctggtgctgcagcttattatgtgggttaagtaggacttcgattggatggaataaaatataatgaaaatggaaccattacagatgctgtagactgtgcacttgaccct

SEQ ID NO: 610 - DNA, 82 bp, synthetic construct
  misc_feature 1..82: note = source = /note="Description of Artificial Sequence: Synthetic oligonucleotide"
  source 1..82: mol_type = other DNA
tctggttactgccagttgaatctgagggtccggacggatatcgcactaagtgtacctggtgcatttcgctgattttggggtc

SEQ ID NO: 611 - DNA, 82 bp, synthetic construct
  misc_feature 1..82: note = source = /note="Description of Artificial Sequence: Synthetic oligonucleotide"
  source 1..82: mol_type = other DNA
tctggttactgccagttgaatctgagggtcccatgaccatgtcactggctacactgaggtgcatttcgctgattttggggtc

SEQ ID NO: 612 - DNA, 82 bp, synthetic construct
  misc_feature 1..82: note = source = /note="Description of Artificial Sequence: Synthetic oligonucleotide"
  source 1..82: mol_type = other DNA
tctggttactgccagttgaatctgagggtccttgacatggcatgtgactccactgtcggtgcatttcgctgattttggggtc

SEQ ID NO: 613 - DNA, 82 bp, synthetic construct
  misc_feature 1..82: note = source = /note="Description of Artificial Sequence: Synthetic oligonucleotide"
  source 1..82: mol_type = other DNA
tctggttactgccagttgaatctgagggtccacctttgccagatgactgagtggaagggtgcatttcgctgattttggggtc

SEQ ID NO: 614 - DNA, 82 bp, synthetic construct
  misc_feature 1..82: note = source = /note="Description of Artificial Sequence: Synthetic oligonucleotide"
  source 1..82: mol_type = other DNA
tctggttactgccagttgaatctgagggtccagcttgaagcgttcgcgacaagtgtcggtgcatttcgctgattttggggtc

SEQ ID NO: 615 - DNA, 82 bp, synthetic construct
  misc_feature 1..82: note = source = /note="Description of Artificial Sequence: Synthetic oligonucleotide"
  source 1..82: mol_type = other DNA
tctggttactgccagttgaatctgagggtcctcacgtcctgagatcaactgctacatggtgcatttcgctgattttggggtc

SEQ ID NO: 616 - DNA, 82 bp, synthetic construct
  misc_feature 1..82: note = source = /note="Description of Artificial Sequence: Synthetic oligonucleotide"
  source 1..82: mol_type = other DNA
tctggttactgccagttgaatctgagggtccgttgactgatcacatgctgctccacgggtgcatttcgctgattttggggtc

SEQ ID NO: 617 - DNA, 82 bp, synthetic construct
  misc_feature 1..82: note = source = /note="Description of Artificial Sequence: Synthetic oligonucleotide"
  source 1..82: mol_type = other DNA
tctggttactgccagttgaatctgagggtcccagacagtcatcggattgatgagtgaggtgcatttcgctgattttggggtc

SEQ ID NO: 618 - DNA, 26 bp, synthetic construct
  misc_feature 1..26: note = source = /note="Description of Artificial Sequence: Synthetic oligonucleotide"
  source 1..26: mol_type = other DNA
tatcttcaacctaggacttttctatt

SEQ ID NO: 619 - DNA, 26 bp, synthetic construct
  misc_feature 1..26: note = source = /note="Description of Artificial Sequence: Synthetic oligonucleotide"
  source 1..26: mol_type = other DNA
atagaacaacctaggacttttctatt

SEQ ID NO: 620 - DNA, 92 bp, synthetic construct
  modified_base 30..39: mod_base = OTHER; note = a, c, t, g, unknown or other
  variation 67..72: note = /replace="atagaa"
  misc_feature 1..92: note = /note="Variant positions given in the sequence have no preference with respect to those in the annotations for variant positions"
  misc_feature 1..92: note = source = /note="Description of Artificial Sequence: Synthetic oligonucleotide"
  source 1..92: mol_type = other DNA
aatgatacggcgaccaccgagatctacacnnnnnnnnnngctggtgctgcagcttattatgtgggttatcttcaacctaggacttttctatt

SEQ ID NO: 621 - DNA, 62 bp, synthetic construct
  modified_base 29..38: mod_base = OTHER; note = a, c, t, g, unknown or other
  misc_feature 1..62: note = source = /note="Description of Artificial Sequence: Synthetic oligonucleotide"
  source 1..62: mol_type = other DNA
agatgctgtagactgtgcacttgaccctnnnnnnnnnnatctcgtatgccgtcttctgcttg

SEQ ID NO: 622 - DNA, 28 bp, synthetic construct
  misc_feature 1..28: note = source = /note="Description of Artificial Sequence: Synthetic primer"
  source 1..28: mol_type = other DNA
agatgctgtagactgtgcacttgaccct

SEQ ID NO: 623 - DNA, 27 bp, synthetic construct
  misc_feature 1..27: note = source = /note="Description of Artificial Sequence: Synthetic primer"
  source 1..27: mol_type = other DNA
acccacataataagctgcagcaccagc

SEQ ID NO: 624 - DNA, 138 bp, synthetic construct
  modified_base 30..39: mod_base = OTHER; note = a, c, t, g, unknown or other
  variation 63..67: note = /replace="gcgtc"
  modified_base 105..114: mod_base = OTHER; note = a, c, t, g, unknown or other
  misc_feature 1..138: note = /note="Variant positions given in the sequence have no preference with respect to those in the annotations for variant positions"
  misc_feature 1..138: note = source = /note="Description of Artificial Sequence: Synthetic polynucleotide"
  source 1..138: mol_type = other DNA
aatgatacggcgaccaccgagatctacacnnnnnnnnnngagcggctgtctccacaagtccgcgcagagccttcaggtcagaacccgctcgcaggtccaaatctnnnnnnnnnnatctcgtatgccgtcttctgcttg

SEQ ID NO: 625 - DNA, 23 bp, synthetic construct
  misc_feature 1..23: note = source = /note="Description of Artificial Sequence: Synthetic primer"
  source 1..23: mol_type = other DNA
gagcggctgtctccacaagtccg

SEQ ID NO: 626 - DNA, 22 bp, synthetic construct
  misc_feature 1..22: note = source = /note="Description of Artificial Sequence: Synthetic primer"
  source 1..22: mol_type = other DNA
acccgctcgcaggtccaaatct

SEQ ID NO: 627 - DNA, 23 bp, synthetic construct
  misc_feature 1..23: note = source = /note="Description of Artificial Sequence: Synthetic primer"
  source 1..23: mol_type = other DNA
cggacttgtggagacagccgctc

SEQ ID NO: 628 - DNA, 108 bp, Severe acute respiratory syndrome coronavirus 2
  source 1..108: mol_type = other DNA
gctggtgctgcagcttattatgtgggttatcttcaacctaggacttttctattaaaatataatgaaaatggaaccattacagatgctgtagactgtgcacttgaccct

SEQ ID NO: 629 - DNA, 108 bp, synthetic construct
  misc_feature 1..108: note = source = /note="Description of Artificial Sequence: Synthetic polynucleotide"
  source 1..108: mol_type = other DNA
gctggtgctgcagcttattatgtgggtatagaacaacctaggacttttctattaaaatataatgaaaatggaaccattacagatgctgtagactgtgcacttgaccct

SEQ ID NO: 630 - DNA, 108 bp, synthetic construct
  misc_feature 1..108: note = source = /note="Description of Artificial Sequence: Synthetic polynucleotide"
  source 1..108: mol_type = other DNA
gctggtgctgcagcttattatgtgggttggactacctaggactgcgcgactaaaaaatataatgaaaatggaaccattacagatgctgtagactgtgcacttgaccct

SEQ ID NO: 631 - DNA, 108 bp, synthetic construct
  misc_feature 1..108: note = source = /note="Description of Artificial Sequence: Synthetic polynucleotide"
  source 1..108: mol_type = other DNA
gctggtgctgcagcttattatgtgggtcacctcgtaggacttctgaaatagccaaaatataatgaaaatggaaccattacagatgctgtagactgtgcacttgaccct

SEQ ID NO: 632 - DNA, 108 bp, synthetic construct
  misc_feature 1..108: note = source = /note="Description of Artificial Sequence: Synthetic polynucleotide"
  source 1..108: mol_type = other DNA
gctggtgctgcagcttattatgtgggtgcttggtggatctcagaacgcggcggaaaatataatgaaaatggaaccattacagatgctgtagactgtgcacttgaccct